European Patent Specification EP 3 778 866 B1, published May 29, 2024. Title: Recombinant yeast strain for producing nervonic acids and application thereof. Applicant: QINGDAO INSTITUTE OF BIOENERGY AND BIOPROCESS TECHNOLOGY, CHINESE ACADEMY OF SCIENCES ZHEJIANG ZHENYUAN PHARMACEUTICAL CO., LTD. The sequence listing filed with the application follows.

SEQUENCE LISTING (127 sequences)

SEQ ID NO: 1 - DNA, 44 bp, artificial sequence
  primer
actttttgcagtactaaccgcagactatcgactcacaatactac

SEQ ID NO: 2 - DNA, 41 bp, artificial sequence
  primer
gcaagaccggcaacgtggggttactcaatcattcggaactc

SEQ ID NO: 3 - DNA, 43 bp, artificial sequence
  primer
catagcacgcgtgtagatacctaagcagccatgccagacatac

SEQ ID NO: 4 - DNA, 42 bp, artificial sequence
  primer
gaattaaacacacatcaacaatggtgaaaaacgtggaccaag

SEQ ID NO: 5 - DNA, 45 bp, artificial sequence
  primer
actttttgcagtactaaccgcagatgagaatctctctactttgtg

SEQ ID NO: 6 - DNA, 40 bp, artificial sequence
  primer
gcaagaccggcaacgtggggtcagttgtagcagtaattgc

SEQ ID NO: 7 - DNA, 44 bp, artificial sequence
  primer
actttttgcagtactaaccgcagatgcaattacggttgattttg

SEQ ID NO: 8 - DNA, 42 bp, artificial sequence
  primer
gcaagaccggcaacgtggggttagttaaaacagtagcggttg

SEQ ID NO: 9 - DNA, 45 bp, artificial sequence
  primer
actttttgcagtactaaccgcagatgaaattctctccacttttgc

SEQ ID NO: 10 - DNA, 43 bp, artificial sequence
  primer
gcaagaccggcaacgtggggttacataagaagagcggcaaaac

SEQ ID NO: 11 - DNA, 45 bp, artificial sequence
  primer
actttttgcagtactaaccgcagatgaagttctcggctaccattc

SEQ ID NO: 12 - DNA, 42 bp, artificial sequence
  primer
gcaagaccggcaacgtggggttagttgtaacagtagtcggag

SEQ ID NO: 13 - DNA, 45 bp, artificial sequence
  primer
actttttgcagtactaaccgcagatcgcaaacttcctgctgcttc

SEQ ID NO: 14 - DNA, 48 bp, artificial sequence
  primer
gcaagaccggcaacgtggggttaaccagagtactgatagcagtattcc

SEQ ID NO: 15 - DNA, 44 bp, artificial sequence
  primer
actttttgcagtactaaccgcagatgcagtttacgcccttattc

SEQ ID NO: 16 - DNA, 46 bp, artificial sequence
  primer
gcaagaccggcaacgtggggtcatttacttgaatcaacacaatatc

SEQ ID NO: 17 - DNA, 40 bp, artificial sequence
  primer
actttttgcagtactaaccgcaggcttctatcccccatta

SEQ ID NO: 18 - DNA, 43 bp, artificial sequence
  primer
gcaagaccggcaacgtggggctatctcatggtcaccagctcct

SEQ ID NO: 19 - DNA, 40 bp, artificial sequence
  primer
actttttgcagtactaaccgcagtccgccgagaaaaccaa

SEQ ID NO: 20 - DNA, 42 bp, artificial sequence
  primer
gcaagaccggcaacgtggggttagggctttttgaggagggtc

SEQ ID NO: 21 - DNA, 40 bp, artificial sequence
  primer
gaattaaacacacatcaacaatggagtctggacctatgcc

SEQ ID NO: 22 - DNA, 41 bp, artificial sequence
  primer
catagcacgcgtgtagatacctactgggcctttttttgagc

SEQ ID NO: 23 - DNA, 41 bp, artificial sequence
  primer
catagcacgcgtgtagatacttaagatcggccgttctgcac

SEQ ID NO: 24 - DNA, 41 bp, artificial sequence
  primer
gaattaaacacacatcaacaatgacctctgtgaacgtgaag

SEQ ID NO: 25 - DNA, 44 bp, artificial sequence
  primer
actttttgcagtactaaccgcagacctctgtgaacgtgaagctg

SEQ ID NO: 26 - DNA, 41 bp, artificial sequence
  primer
gcaagaccggcaacgtggggttaagatcggccgttctgcac

SEQ ID NO: 27 - DNA, 44 bp, artificial sequence
  primer
actttttgcagtactaaccgcagacctctatcaacgtgaagctg

SEQ ID NO: 28 - DNA, 40 bp, artificial sequence
  primer
gcaagaccggcaacgtggggttaagatcggccgttttggg

SEQ ID NO: 29 - DNA, 44 bp, artificial sequence
  primer
actttttgcagtactaaccgcagaacatgtctgtgctgaccctg

SEQ ID NO: 30 - DNA, 40 bp, artificial sequence
  primer
gcaagaccggcaacgtggggttactcggccttggtggcct

SEQ ID NO: 31 - DNA, 47 bp, artificial sequence
  primer
actttttgcagtactaaccgcagatcatcaagaacaacaacaacggc

SEQ ID NO: 32 - DNA, 42 bp, artificial sequence
  primer
gcaagaccggcaacgtggggttagtctcgcttggtgggcttc

SEQ ID NO: 33 - DNA, 43 bp, artificial sequence
  primer
actttttgcagtactaaccgcagtctgtgctgaccctgcagga

SEQ ID NO: 34 - DNA, 40 bp, artificial sequence
  primer
gcaagaccggcaacgtggggttagtcggccttggtggcct

SEQ ID NO: 35 - DNA, 43 bp, artificial sequence
  primer
actttttgcagtactaaccgcagtcctccgtggtcgagacctg

SEQ ID NO: 36 - DNA, 46 bp, artificial sequence
  primer
gcaagaccggcaacgtggggttaacccagaataccctcagagtcag

SEQ ID NO: 37 - DNA, 44 bp, artificial sequence
  primer
actttttgcagtactaaccgcagaccgtcaagacccgatccaac

SEQ ID NO: 38 - DNA, 50 bp, artificial sequence
  primer
gcaagaccggcaacgtggggttacataatagatttacctcgctggatgtc

SEQ ID NO: 39 - DNA, 43 bp, artificial sequence
  primer
actttttgcagtactaaccgcaggccacccccctgcctcctac

SEQ ID NO: 40 - DNA, 45 bp, artificial sequence
  primer
gcaagaccggcaacgtggggttactcctccttagagtggtcgccg

SEQ ID NO: 41 - DNA, 44 bp, artificial sequence
  primer
actttttgcagtactaaccgcagtctctgtctgcctctgagaag

SEQ ID NO: 42 - DNA, 40 bp, artificial sequence
  primer
gcaagaccggcaacgtggggttatcggaccatggccattc

SEQ ID NO: 43 - DNA, 44 bp, artificial sequence
  primer
actttttgcagtactaaccgcagtctgtgacctctaccgtggag

SEQ ID NO: 44 - DNA, 40 bp, artificial sequence
  primer
gcaagaccggcaacgtggggtcatctcacgatggccattc

SEQ ID NO: 45 - DNA, 44 bp, artificial sequence
  primer
actttttgcagtactaaccgcagaattttcatcatctggcttac

SEQ ID NO: 46 - DNA, 42 bp, artificial sequence
  primer
gcaagaccggcaacgtggggtcaggcctccaggcttatccag

SEQ ID NO: 47 - DNA, 40 bp, artificial sequence
  primer
actttttgcagtactaaccgcagagtgaaggccccgtcaa

SEQ ID NO: 48 - DNA, 43 bp, artificial sequence
  primer
gcaagaccggcaacgtggggctaattatccttcgtatcttctg

SEQ ID NO: 49 - DNA, 40 bp, artificial sequence
  primer
tctcaagggcatcggtcgaccaacttttcttgtcgacctg

SEQ ID NO: 50 - DNA, 32 bp, artificial sequence
  primer
cacgctccatttagcgtgtcgtgtttttgttg

SEQ ID NO: 51 - DNA, 40 bp, artificial sequence
  primer
tctcaagggcatcggtcgacagagaccgggttggcggcgc

SEQ ID NO: 52 - DNA, 41 bp, artificial sequence
  primer
caacgtggggctgcggttagtactgcaaaaagtgctggtcg

SEQ ID NO: 53 - DNA, 40 bp, artificial sequence
  primer
tctcaagggcatcggtcgacaaggagtttggcgcccgttt

SEQ ID NO: 54 - DNA, 37 bp, artificial sequence
  primer
cacgctccattgctgtagatatgtcttgtgtgtaagg

SEQ ID NO: 55 - DNA, 39 bp, artificial sequence
  primer
tctcaagggcatcggtcgactttgtgcaagtgtgtgtgt

SEQ ID NO: 56 - DNA, 30 bp, artificial sequence
  primer
cacgctccatagtagatgtgtaagtgtgta

SEQ ID NO: 57 - DNA, 40 bp, artificial sequence
  primer
tctcaagggcatcggtcgaccgcagtaggatgtcctgcac

SEQ ID NO: 58 - DNA, 46 bp, artificial sequence
  primer
gtgtagatactgttgatgtgtgtttaattcaagaatgaatatagag

SEQ ID NO: 59 - DNA, 30 bp, artificial sequence
  primer
ctaaccgcagccccacgttgccggtcttgc

SEQ ID NO: 60 - DNA, 41 bp, artificial sequence
  primer
gctgtcaaacatgagaattcggacacgggcatctcacttgc

SEQ ID NO: 61 - DNA, 30 bp, artificial sequence
  primer
cacatcaacagtatctacacgcgtgctatg

SEQ ID NO: 62 - DNA, 44 bp, artificial sequence
  primer
gctgtcaaacatgagaattcctaccttgctcgaatgacttattg

SEQ ID NO: 63 - DNA, 31 bp, artificial sequence
  primer
atctacagcaatggagcgtgtgttctgagtc

SEQ ID NO: 64 - DNA, 38 bp, artificial sequence
  primer
gctgtcaaacatgagaattcatttcttgacctcatcaa

SEQ ID NO: 65 - DNA, 49 bp, artificial sequence
  primer
ctcacatcacatccgaacataaacaaccatgaaaaagcctgaactcacc

SEQ ID NO: 66 - DNA, 48 bp, artificial sequence
  primer
acaagaatctttttattgtcagtactgactattcctttgccctcggac

SEQ ID NO: 67 - DNA, 41 bp, artificial sequence
  primer
tacaaccacacacatccacaatggaacccgaaactaagaag

SEQ ID NO: 68 - DNA, 40 bp, artificial sequence
  primer
agggccctttttatagagtcttatacactagcggaccctg

SEQ ID NO: 69 - DNA, 40 bp, artificial sequence
  primer
tacaaccacacacatccacaatgccctcctacgaagctcg

SEQ ID NO: 70 - DNA, 48 bp, artificial sequence
  primer
agggccctttttatagagtcctaacagttaatcttctggtaagcctcc

SEQ ID NO: 71 - DNA, 21 bp, artificial sequence
  primer
aattccgtcgtcgcctgagtc

SEQ ID NO: 72 - DNA, 21 bp, artificial sequence
  primer
gtcgaccgatgcccttgagag

SEQ ID NO: 73 - DNA, 46 bp, artificial sequence
  primer
tctcaagggcatcggtcgaccccggggtggtaatcgaccgactaac

SEQ ID NO: 74 - DNA, 41 bp, artificial sequence
  primer
actcaggcgacgacggaatttgacgaggtctggatggaagg

SEQ ID NO: 75 - DNA, 22 bp, artificial sequence
  primer
gatctcggcagtctctcggatg

SEQ ID NO: 76 - DNA, 20 bp, artificial sequence
  primer
tgttcggaaatcaacggatg

SEQ ID NO: 77 - DNA, 40 bp, artificial sequence
  primer
catccgttgatttccgaacatttgagccgaggcagatttg

SEQ ID NO: 78 - DNA, 47 bp, artificial sequence
  primer
tccgagagactgccgagatccccgggtcagagagaaggactatggag

SEQ ID NO: 79 - DNA, 38 bp, artificial sequence
  primer
gaattctcatgtttgacagcttatcatcgatgataagc

SEQ ID NO: 80 - DNA, 21 bp, artificial sequence
  primer
gtcgaccgatgcccttgagag

SEQ ID NO: 81 - DNA, 20 bp, artificial sequence
  primer
ccccacgttgccggtcttgc

SEQ ID NO: 82 - DNA, 22 bp, artificial sequence
  primer
ctgcggttagtactgcaaaaag

SEQ ID NO: 83 - DNA, 1545 bp, Yarrowia lipolytica
  Yarrowia lipolytica DGAT1
atgactatcgactcacaatactacaagtcgcgagacaaaaacgacacggcacccaaaatcgcgggaatccgatatgccccgctatcgacaccattactcaaccgatgtgagaccttctctctggtctggcacattttcagcattcccactttcctcacaattttcatgctatgctgcgcaattccactgctctggccatttgtgattgcgtatgtagtgtacgctgttaaagacgactccccgtccaacggaggagtggtcaagcgatactcgcctatttcaagaaacttcttcatctggaagctctttggccgctacttccccataactctgcacaagacggtggatctggagcccacgcacacatactaccctctggacgtccaggagtatcacctgattgctgagagatactggccgcagaacaagtacctccgagcaatcatctccaccatcgagtactttctgcccgccttcatgaaacggtctctttctatcaacgagcaggagcagcctgccgagcgagatcctctcctgtctcccgtttctcccagctctccgggttctcaacctgacaagtggattaaccacgacagcagatatagccgtggagaatcatctggctccaacggccacgcctcgggctccgaacttaacggcaacggcaacaatggcaccactaaccgacgacctttgtcgtccgcctctgctggctccactgcatctgattccacgcttcttaacgggtccctcaactcctacgccaaccagatcattggcgaaaacgacccacagctgtcgcccacaaaactcaagcccactggcagaaaatacatcttcggctaccacccccacggcattatcggcatgggagcctttggtggaattgccaccgagggagctggatggtccaagctctttccgggcatccctgtttctcttatgactctcaccaacaacttccgagtgcctctctacagagagtacctcatgagtctgggagtcgcttctgtctccaagaagtcctgcaaggccctcctcaagcgaaaccagtctatctgcattgtcgttggtggagcacaggaaagtcttctggccagacccggtgtcatggacctggtgctactcaagcgaaagggttttgttcgacttggtatggaggtcggaaatgtcgcccttgttcccatcatggcctttggtgagaacgacctctatgaccaggttagcaacgacaagtcgtccaagctgtaccgattccagcagtttgtcaagaacttccttggattcacccttcctttgatgcatgcccgaggcgtcttcaactacgatgtcggtcttgtcccctacaggcgacccgtcaacattgtggttggttcccccattgacttgccttatctcccacaccccaccgacgaagaagtgtccgaataccacgaccgatacatcgccgagctgcagcgaatctacaacgagcacaaggatgaatatttcatcgattggaccgaggagggcaaaggagccccagagttccgaatgattgagtaa

SEQ ID NO: 84 - DNA, 1449 bp, Yarrowia lipolytica
  gene SCD
atggtgaaaaacgtggaccaagtggatctctcgcaggtcgacaccattgcctccggccgagatgtcaactacaaggtcaagtacacctccggcgttaagatgagccagggcgcctacgacgacaagggccgccacatttccgagcagcccttcacctgggccaactggcaccagcacatcaactggctcaacttcattctggtgattgcgctgcctctgtcgtcctttgctgccgctcccttcgtctccttcaactggaagaccgccgcgtttgctgtcggctattacatgtgcaccggtctcggtatcaccgccggctaccaccgaatgtgggcccatcgagcctacaaggccgctctgcccgttcgaatcatccttgctctgtttggaggaggagctgtcgagggctccatccgatggtgggcctcgtctcaccgagtccaccaccgatggaccgactccaacaaggacccttacgacgcccgaaagggattctggttctcccactttggctggatgctgcttgtgcccaaccccaagaacaagggccgaactgacatttctgacctcaacaacgactgggttgtccgactccagcacaagtactacgtttacgttctcgtcttcatggccattgttctgcccaccctcgtctgtggctttggctggggcgactggaagggaggtcttgtctacgccggtatcatgcgatacacctttgtgcagcaggtgactttctgtgtcaactcccttgcccactggattggagagcagcccttcgacgaccgacgaactccccgagaccacgctcttaccgccctggtcacctttggagagggctaccacaacttccaccacgagttcccctcggactaccgaaacgccctcatctggtaccagtacgaccccaccaagtggctcatctggaccctcaagcaggttggtctcgcctgggacctccagaccttctcccagaacgccatcgagcagggtctcgtgcagcagcgacagaagaagctggacaagtggcgaaacaacctcaactggggtatccccattgagcagctgcctgtcattgagtttgaggagttccaagagcaggccaagacccgagatctggttctcatttctggcattgtccacgacgtgtctgcctttgtcgagcaccaccctggtggaaaggccctcattatgagcgccgtcggcaaggacggtaccgctgtcttcaacggaggtgtctaccgacactccaacgctggccacaacctgcttgccaccatgcgagtttcggtcattcgaggcggcatggaggttgaggtgtggaagactgcccagaacgaaaagaaggaccagaacattgtctccgatgagagtggaaaccgaatccaccgagctggtctccaggccacccgggtcgagaaccccggtatgtctggcatggctgcttag

SEQ ID NO: 85 - DNA, 1647 bp, Yarrowia lipolytica
  gene PLA2-1
atgagaatctctctactttgtgttgcaactctttgcagctctgtcttggccctctacacaccccaacgtggaacatgtccttcttcacctctacttcgacaagccaagggacttcaaagcgatgaagcagagtacatgtccagccgtcggaacaagaccaaacctgccttgagtacctttctgaaaaagcaaaacattgacaatttcgatgtcgattccttcctcgaacgggcgtcccccaagttggctgtggctgccgctggaggaggcctgagagccacttatatgggcatgggtacattccaggcactcgacaaccgaacagagaactccactcttgccggttacctccaggccgtcgactacatgtcgggattgtctgggggttcgtggctagtaggctacctagctatcaacgattatccagatttccagactcttttccacgcgtttgacggcattttcaatcttccaggatccatgggaactctgggaatgctagctaaagtgttcattgactcccttcagaaactcaaggctggttatcagacgtcggtcactgaccagtggggaagacttatctacctgttgttgggcaacgctgggctgctaaaagcagattttaattggtcggacatccgaaatctgacctccttcacatctcatgaaatgcccttccccatcattcttggtaccactgtttttcccggctcttctttcgacgtggagtacataacctataacaactcgatcatggaaatgactccatatgagttcggaacatgggacaaaaacatccgggagttcatcgacatgcagtatctgggcactgaaatggaaaacggcacccccgtgggtgaatgtaccaccaattacgacaacgccggccttctgatgggcatttcttccaacgtgttcaatgcgggtctagacggacttggaatcgacggaatttttggaatcttggtcgaagatcttatgaaactgctggaaatcatcaacgacgcctcttaccgcctcggtgtcatttctcctaacccgttctacaagcaggatgacattccttcgaaccagaccatctccagaggtctactagtgtgtgacggaggctttgatctcgaaactatccccatcctgccctttttgcaacccgaacgagaagttgatgttgtcatctccatggatccttctctagacagccccgagggatggcccactggagaatgtatcagacataccgcagccaaaagtcaatgggagtttggagagggagtgttcccccagattcccgacaatgtcaccttcatcaacgacaacctcaccaccaagcctgtcttctttggttgcaacatcaccaacctgaagaagtacgataacaccgacagatactctccggtcatcgtctacgtacccatgcacaacatttcctacgtgtccaacttctccactggaaagctcttgtataccaaggaggaaagcttcggaaccgtcaacaatgcgtacaacatgatgacaaggacaaacttgaccgaagatgaagaatggggcaaatgcctaggttgcgtttccattctccgagagctgcagagattgaatgagaccgtgccggattgtgagaggtgtttcagcaattactgctacaactga

SEQ ID NO: 86 - DNA, 1653 bp, Yarrowia lipolytica
  gene PLA2-2
atgcaattacggttgattttgacggcatttgcctctttggcaattgcagactacactcctgtgcgagttccatgtccctccaccaatcttacgcgtcctgccattggactgaatcctgacgaatctgcttacattgagcagcgacataccaagaccagagaaagcctcaagacatttctgaagactctagaaagttcctcttttgatgttgatgcctttctgaatgagaggtctcccaagatcgccgttgcaattgctggaggaggagtaagagcttctctgtttggagccggagttttggctggtctggatggtcgagtttcccaaaacggtaccgggggtctgcttcaggcaacagactacatttctggtctttctgggggctcctggcttgttggactgctctgtttgtctgactggatagccgctgaccagctagttggaatgagcgagaaaatgaagttcccaggcatgcttgacacttttggcatgatgctcaagattctcacagacaccatggctaagaaaaaggccggctaccagacatccgtggttgatcagtggggcagactgttccattttgtgactgccgaagctggtttgaactacacggatccgacatggagtggaattcgcaacctgagctcgttcctggacttctccatgccctttcctataatcacctcaacttctttatttccaggaacctcgtttgacgtcacccatatcgactatatcaaccccatggttgaaatgacacccttcgagttcggaagctgggacagaaacttccgttacttcgctgacactgtgtttctgggcacggagatggaagacgcgaagcccctgaatcagtgtgtgcgtaattacgacaatcacggtctattcctgggttcttcaggtggaatcttcaatgctgacgtgatcggcggatttgaaatgaaaggcttacatgcgatatttttgtctggagtcttggagtatcttgatcttgtcaacgaaggtgagttccgagtaggacttattcagaaccccttctacaagatggcacatctagtctccaaccagacaatctccaggttcatgtacttgtgcgatggagggtttgagaagcaacaaaacattcctttgcttccttttcttcagcctgaacgagaaatagatcttctctttgccactgatccatcaacagatactatggatggtcatggatggcccaatggagcttctctgagacacacaaaggagaagagtgacctggagtttggcaaaggaatttaccctgaaattcccgaggaggacgagtacttgagcagaaacttgtccatgcaacctgccttctttggctgcgatatcgcttctctgaaacagtacaacaatacgcaacggtatgcccctgtgattgtcaacattcccatgggaaacctgacgtatgcttcgaatttctcgactggtaagttcttttacactcatgaagaaacccagggaacctatttgaatgcctacaatatggccactaggtccaacttgaccgaggacgagaattggaacgtgtgtctagggtgcgtatcactgttgcgcgaatttcagagacggtccagtgaaatccccgaccaatgtcagacctgcttcaaccgctactgttttaactaa

SEQ ID NO: 87 - DNA, 1917 bp, Yarrowia lipolytica
  gene PLA2-3
atgaaattctctccacttttgctggcgaccgtgggtctggcccagagcttctattcgcccaccgactcgtacgcgcccgggtcggtcgactgtccctccaactccacccagattgtgcgaaagggcgagggcctttcttcgcaggaacgagagtgggtccagaaccgacacgaacagacccgaccggagctgctcaactacctgaaacgggtgggctttaagtcggtggacccggaccagttcctgggccaggacactaatatcaccatcggactgtccttttctggaggaggatacagagccatgttggcgggagcaggccaatttgcggctctggacgcgcgaacacccaacgccaccgaaccgggccatgtgggaggtctggtccaggccgccacctatctggtgggtctttcgggcggaaactggatggtgggatctgtggtcatcaacaacttcaccaccattcccgacctgcaacactcgtccgacgtgtgggacctggaacactccatgatcaaccccggcggaatcaacatcttcaagaccggctcttattgggacgacatcaacgacgacgtcaacgacaagcagcacgccggatacaacacctctttcaccgacatctggggccgaggtctgtcgtaccagttcttcaacgcttccaacaccgcccgactcacctggtccgagatccagaactacgaccacttcaagaaccactctatgccctaccccattgttgtggccgacggccgagcccccggaacccgaatcatctccggaaactccaccattttcgagctggccccgttcgaggtcggctcctgggaccccaatgtctactcctttgccaagaccgagtggctgggaaccaacatgaccaacggccgacccaacggaacctgtgtgcatggctttgacaacgccggtttcattgtgggaacctcttcttccctgttcaaccagttcattctccagctcaactccaccggagtaaccggagtggtctacgacctggcccactctatcctcaagcgtctggataaggactcggacgatatcgccatctactcgcccaaccccttcaagggcatgtcctacctcggcaactcgtccattgcccaaaccgagtatctggatctggtcgacggaggagaagatggacagaatgtgccctactaccctctgctgcagcccgagagagccgtcgacgtggtcatctcctacgacaactccgccgacaccgactttaactggcccaacggaacctccgctgtccagacataccgacgacagtttgagaaccaggccaatggcaccattttcccctacgtgcccgacgtgaacacattcatcaatgagaacctgacttctcgacccgccttctttggctgtgacgtgcagaacatgacctcgctggacaagaacggttataccgacgtcaactcttccgccgcccttccccctctcattgtctacattgctaactacccctggacctttttctccaacacatcgaccatgtccaagctgtcgtacaacaagaaggaggttgccggcatgatcgagaacggctactccacctccacccagttcaacggaaccgtggaccccgactggcctgtgtgtcttggctgtgctctgctcaagcgagaggccacccgacgaaaccagtctctgggctctgactgtgacaagtgcttctccaagtactgctggaacggaaagactgacgatgatgccgaaaaggctctgaagtttgctcccgccatctatgccaacggccctaacgtttcttccaacgcctcaattggccaggcttcgtccacctccaagcccaagaagaacggcgccgagggtctggttccgggtatggctgccattgccattggttttgccgctcttcttatgtaa

SEQ ID NO: 88 - DNA, 1710 bp, Yarrowia lipolytica
  gene PLA2-4
atgaagttctcggctaccattctgaccgccctggcagcctcggcggttgccaactacgcccccatcaaggtggagtgtccaaaagatgtcaacatctcccgaccagcagacggcctgagccaccaggaggccgactacatcaatgaacgacacaaaaagacctccaaggcgctcagagagtacctcggtgggctcgacatcaaggcccgaggcaacaacaccttcgacacggactcttttctgaacgaaacctcccccaagctcgccattgcggctgccggaggaggtttccgggccatgctggttggagcaggcgtcattgctgccctggacaagcgtgtggacgaaaacaacaagaacggaggctttctgcagtccgcagactatctggccggtttgtctggaggagcttggctcgtgggatctctggtcctcaacgactggcctactgtgcctgagatccaggctgacccccaaatctggtacctcaacaagtccttggtgggctcagtcgaacccggatccatgaacaccgtcggcctcttcgccaaggtgcttgcagataccacctccaagcttgctgccggctaccagacctcgctgaccgaccaatggggacgactggtgtcataccagaccatcaactcttcgcacaccaagggcggtctggatgccaccgaggtgacctggtctggcatcagaaacatctcctctttcgttgaccatgaaatgccctttcccatcattctgggcacatctcttttccccggaacttctcacgatgttgaccagattaaattcaacaactccatcatcgaaatgaccccctacgagtggggaacctgggacaagaacatccggcaatttgtcgacaccgagtacctgggtaccgagatgtccgacggaaagcccacaggaaactgtacccgacgatacgataacgccggcttcctgatgggaacctcctcctcaattttcaacatggacatgaagactctgggctttggcggctttgagagcgtgctactgcaggatctcttctccgctctggatattgtcaacgagggctctttcaacgtggctgtttacaaccccaaccctttctaccaacaggttggcatgcagaccaatcagaccatctccaaggctctgtacgtgtgtgacggaggtttcgacaaggagaccattcccattctgcctttccttcagcccgagagagaggtcgatgttgtcattgccatcgacccttccactgatactgaggaaagctggcccgatggagagtctcttcgagccacccagaacaagtccgactgggagtttggagacgacgtgtttcccaagatcccctctaacgagaccttcatcagcaagaatctgactaccaagcctgtcttcttcggctgcaacaccaccaatctcaagacgtacaaggactcggatcgatactctcccgtcattgtctacgtgcccatgtctgacatcacctacccctccaacttctccaccggcaagctgtcctacaccaacgaggaacagcagcgaaccatcaacaacggctacaacatgatgactcgaagcaacggaaccgaggattccaactgggacaagtgtctgggctgtgtgactctgctgcgagagttccagcgacgggactcggatgttcccaatgactgtgagcagtgtttctccgactactgttacaactaa

SEQ ID NO: 89 - DNA, 1623 bp, Yarrowia lipolytica
  gene PLA2-5
atgatcgcaaacttcctgctgcttctggtgctggtcaccttcgctgcagcctcctacactccctccaagggaagctgccaatacgacaccaacctgcttcgagaagcctccagtatctctcctgatgaggccaactacgttgcctccaagcagtccagttccgattccgctttccagagctacctcaagaacgtcaacatccctggtctggatgtgaaccagtctgccaacattgccctttccttctctggaggaggatatcgagctatgttgtccggtgctggccaattttctgctctggatagccgaaacgagatcgccaacactatgggaggtcttttacaggcatccaactatcttgtcggatgctctggaggtggatggctggtcggcactattgccatgaacaacttccctactatcgctgaggtccgatccaactctgacctgtggaagatcaatgacaatgttcccgagcttactaaccctctttcttggttggcgtttggtagatatgctggcattgttactgctgcccttggaaagcgtttggccggatttaaaatctctttcaccgacgagtggggtctgctcgtggggcgaaatcttgttgataagaacggcccatactctacctggtccgacatcaaggtcacccaatcttacctgtccaacgagattcccttccctatcattgtcggtaccactctgaacagcgctgatgagcaggaggctcagattactatcgacaaccctttgattgagatgacccccattgagttcggctccttcgacaagtccatcaaatctttcttcactacttctgctattggtacttctgtttctaacggccagcccacctcttcccgatgtgtcactggcttcgacaatgcccagttcctgctgggaaccacatccagtcttttccagggtgtcagtggatggcagaagactatgctgaacattgttggggctcttaacggcaacatcgcacccagtgccatctatcaccccaaccctttcaaggatgccagctcggtccaggctcctttcaacggtgactctctctatgcttcagacggaggttattctggcatggttcttcccctgtggccccttatgcagccatctcgaaacgtggacttggtattctcattcgataacagcgcaggaggtcccaacaatgctcctagtggagtcactctggctaacgtgaagcagaaggtcacaaacgagatgggcgaaggagtgttccccgaggttcccagcagcgaggagtacattgccaactaccttgtcaagccagtgtggctcggatgtgaagtttccaagctcaaaaaaatccccaacacagatcgatacgttcctcttgtcatcacaatggccaaccaccagatcaactacaactctcttcagcagactgacaagatggactatagctctgatgagcaaactggtatgatctctaacggttttgcagtcgcttctaacaatggtgacctgaagtgggcccagtgtgtcggctgtgcgggtattctccgagagttccagagaactggtaaggaactccctgaaacctgccaggcttgtctcaaggaatactgctatcagtactctggttaa

SEQ ID NO: 90 - DNA, 3009 bp, Yarrowia lipolytica
  gene PLA2-6
atgcagtttacgcccttattcctgcatttggtggccactcttgccgcttcccctggcggcacatatgagcccaaacatgttgattgtcccccaaccgtactggttcgagaggccaacgataccctcaatcccaaagagaaagactacatggaccggcgatggctgcagactcagcaagaacatgtcaagtttatggaacgtctcgacattcccgacttcaacgtctccttcttggacgaagtcccccctgtcgtgatgggaactgccttctctggaggtggttatcgatccatgttgacaggagcaggtgtcgttgctgccatggacgcccgtgtaaacgggtctcttgaccttggcgcgctgggtggtctcttccaagcaatgtcctacttggtgggcttgtccagtggaagttggttgttgacctctctctttctgaacgacaacttcactgttcctgaccttcaggctgctcctaacctctggagtctcgagaactcattctggggtggagaacgaatgaaggacgtccagcttgacaaccccgttcccaaccctggtattattgataacaacggaaccgagagtgacaacagttctcttgtcattggatctggcctgacagatcgtctgagctctcgactgaagaatctcgtcaatctagctcctcggaacatcgtttccgactcaatcaagcaccactggaatcgacgaccttcgaccggtggagctgaggttgtcaaaaacattaacctcaacgacatgttggccaaacgacctaactctggtatcgctgagcgtcttcgaaacatgcctccaatcggtgagagcatttccaatggtcggcgtactcgtcctagcactggttttgctgaccgtctgagaaacagaccgaagactggaatctctgacagactacaccaccgtcccagtactggactctctgatcggctgcgaaacaggcccagtactggcgtttccgacacctggaagaatcgacccaagactggctatgctgatcggctcaagaattctcaacggccccacttcgatctcgcccaacgactcagaaatagacccaagacaggaatatatgataacgtcgacaaggggatctctcgaataaaacctgggttgtctgatgcccgaaaggctcttgacaaacacattccttcgaaaccttcaatgggtgacttctttaaccagagaagacgtcagtctgatctcgaaaagctcttggagtacgtttctcctgacttcctctgtgacctagactattcagagttcctgaagtaccttgaccctctgtatacttattaccacctggagaatgagatcaagcagaccctgtactacttcctgatgatcaaggaagaggtcgacctgaaatccagtgctggttttgtgaccactatcactgattactggggtcgagcactcgcccgtcagctgcttcctgattctcgaggaggacagggtactacctggtccgatgttcaaatcacacctcagttcatgaacgcatctgtgcctttccctatcatggttgcgattggtcgagagccctccgagtctaacagtacctacatgatctctcctctttggtcgactctcttcgaaatgactcccttcgagtttggatcttggaacccttctttaaacgccttctctgacactcgataccttggttcatccctctataatgggacccccgtcaacaatgttacccttgagcctgttccctcaactgagcccgtttgtgtcttgggatatgataatgctggtttccttgccggcacttcttcctctgtcttcaatgatcctttcgagaattcgggtatcgatcaggactacattcgagagctctttactggtatcattgatgcccttgagaatttcaatacctctttctggggtgaattcttttctacagagaacagcactgtccctgaaactgatcttacttggcgggacgccgactatgccatcttctcacccaaccccttccttgggtttgactctaacgccaccactgataagttttctgagtccaaacatcttttcctggctgatggtggtgaggatggccagctggttcccttcgagcccctacttcaggaacagcgtaatgttgatgtcatcttcgccattgatgcgtcttcgaacactgaggacaacttcccagatggaactgcgctgcgtatgtcacaagagagatacctttcggaggattctgagcaggcggctggcatatcgtttccccagctggctgcagagtttggcaatgaacctgttttccttggatgtttcataaactcgtcttactcggtaccacccaaggggagagcctacagctataactatcgacgagaccgtcctgccgagcccaatatgactattcctgtatatcctcctcctcccccgttcgatttccctaactctacctttgatcctaactccactttttcaaatgttagtatggcttccagggctcactggagagccagacagattcctgtttccaacggcactactaatgatacgggacctataattcgccctcgacctcgccctcgaccccggccctcacgaccccggcctatcatcgaagatggtcgtgactatgacgctgactatccttatgaccacactacccctattggtgccattccagtcatgcctcctacaaatgtttccaccgacccctttgtcaacgttactgttggtgtcgacaagtaccctcctctcattgtgtatatcccaaacagctaccaatcttactggaccggtgatagtactttccaggttgagttttccaccgaggatgttgccggctacattaccaacggctacaatctgatgaccagacagaactccactgtcgaccccgactggaataagtgcgttggttgtgccactattctccgggcttatcagggagccaacaagaccatcccagacttttgcatgggatgtttcgatcgatattgtgttgattcaagtaaatga

SEQ ID NO: 91 - DNA, 1413 bp, Yarrowia lipolytica
  gene ylGSR
atggcttctatcccccattatgactatctggttatcggcggaggctctggaggtgttgcttctgctcgtcgagccgcctcgtacggcgccaaaacactgctgatcgagggcaaggcgctgggaggcacctgcgtcaacgtgggctgtgtgcccaaaaaggtcatgtggaacgcgtccgatctggcgggccgaatccgacaggccaaggagtacggcttccccgacgtggaccccaagtacgccgacaactttgactggtccggattcaaggccaagcgagacgcttacgtcaagcgactcaatggaatctacgaacgaaacctccagaaggagggcgtcgagtacgtgtttggctgggccaccctctacaagcaggagggccaggagttccccctggtacatgtcaagagcgacgacggcaataccaagctgtattctgccaagaagattatgattgccaccggcggaaagccccgtctgcccgacgtgcctggagccgagtacggcattgactccgacggcttctttgctctcgagacccagcccaagcgagtggcggtggttggaggaggctacattggcgtggagctggctggtgtcttccacggactcaactccgagaccaccctcttctgccgaggccagacggtgctccgagcgttcgacatcatgatccaggacaccatcaccgactactacgtcaaggagggcatcaacgtgctcaagggctccggcgtcaagaagattgtcaagaaggacaatggcgagctgctcgtcacctacgagcaggatggcgccgagaaggatatcactcttgactcacttatttggaccattggacgagagcctctcaaggacaccctcaacctcggcgagtttggcatcaagaccaacaagcggggctacattgaggtcgacgagtaccagcgatcgtccgttgacaacatttactcgcttggagacgtttgcggcaaggtcgagctaacccccatggctattgctgccggacgaaagctgtccaaccggctgtttggtcccacagagttcaagaaccagaagcaggactacaccgatgttccttctgccgtcttttcccaccccgaggttggctccatcggtatcaccgaggctgccgccaaggagcagtatggcgaggagaacgtcaaggtctacacctccaagtttgtcgccatgtactacgccatgctcgaggagaaggctcccaccgcctacaagctggtgtgtgccggcaaggacgagaaggttgttggtctgcacattgttggcgctgactctgccgagattctgcagggtttcggcgtggccattcgaatgggagccaccaaggccgatttcgacaatgttgtggctatccatcccacttctgccgaggagctggtgaccatgagatag

SEQ ID NO: 92 - DNA, 507 bp, Yarrowia lipolytica
  gene ylGPO
atgtccgccgagaaaaccaataccgctttctacaacctcgctccactcgacaagaacggagagcctttccccttcaagcagcttgagggcaaggtcgtgctcatcgtgaacgtcgcctccaagtgtggctttactccccaatacaagggccttgaggaggtctaccagaagtacaaggatcagggattcaccatcatcggcttcccctgcaaccagtttggtggccaagagcctggttccgctgacgagatctcctccttctgtcagctgaactacggcgtcactttccccgttcttcagaagatcaacgtcaacggcaacgacgccgaccccgtctacgtctacctgaaggagcagaaggctggtctgctgggcttccgaggaatcaagtggaactttgagaagttcctggttgataagcacggtaacgtcgtcgaccgatatgcttccctcaagacccccgccggcctcgaatccaccatcgagaccctcctcaaaaagccctaa

SEQ ID NO: 93 - DNA, 828 bp, artificial sequence
  gene MaLCE
atggagtctggacctatgcctgccggaattccctttcccgagtactacgacttcttcatggactggaagacccctcttgctatcgctgccacttacactgtggctgtgggcctgtttaaccctaaggtgggcaaggtgtctagagtggtggccaagtctgccaatgctaagcccgccgagagaactcaatctggagccgccatgaccgcttttgtgttcgtgcacaacctgatcctgtgcgtgtactctggcatcaccttctaccacatgttccccgccatggtgaagaacttccgaacccacactctgcacgaggcctattgtgacaccgaccagtctctgtggaacaacgcccttggctattggggctacctgttctacctgtctaagttctacgaggtgatcgacaccatcatcatcatcctgaagggccgacgatcttctctgctgcagacctaccatcatgctggagccatgatcaccatgtggtctggcatcaactaccaggctacccccatctggatcttcgtggtgttcaactctttcatccacaccatcatgtactgctactacgccttcacctctatcggctttcatccccccggcaaaaagtacctgacctctatgcagatcacccagttcctggtgggcattaccatcgccgtgtcttacctgtttgtgcccggctgcatcagaactcctggcgcccaaatggctgtgtggatcaacgtgggctacctgttccctctgacctacctgtttgtggacttcgccaagcgaacctactctaagcgaaccgccatcgccgctcaaaaaaaggcccagtag

SEQ ID NO: 94 - DNA, 1521 bp, artificial sequence
  gene AtFAE1
atgacctctgtgaacgtgaagctgctgtaccgatacgtgctgaccaacttcttcaacctgtgcctgtttcccctgactgcctttcttgccggaaaagcctctcgactgaccatcaacgacctgcacaacttcctgtcttacctgcagcacaacctgatcaccgtgaccctgctgtttgccttcaccgtgttcggactggtgctgtacattgtgacccgacccaaccctgtgtatctggtggactactcttgttacctgcccccccctcaccttaaagtgtctgtgtctaaggtgatggacatcttctaccagatccgaaaggccgacacctcttctagaaacgtggcctgcgacgacccttcttctctggacttcctgcgaaagatccaggagagatctggcctgggcgacgaaacttactctcccgaaggcctgattcatgtgcctccccgaaaaactttcgccgcctctagagaagagaccgagaaggtgattatcggcgccctggagaacctgttcgagaacaccaaggtgaacccccgagagatcggcattctggtggtgaactcttctatgttcaaccccaccccctctctttctgccatggtggtgaacaccttcaagctgcgatctaacatcaagtctttcaacctgggcggcatgggatgttctgctggagtgatcgccatcgacctggctaaggacctgctgcacgtgcacaagaacacctacgccctggtggtgtctaccgagaacatcacccagggcatctacgctggcgagaaccgatctatgatggtgtctaactgcctgttcagagttggaggagccgccattctgctgtctaacaagtctggcgaccgacgacgatctaagtacaagctggtgcacaccgtgcgaactcatactggcgctgacgacaagtctttccgatgcgtgcagcaggaggatgatgagtctggcaagatcggcgtgtgcctgtctaaggacatcaccaacgtggctggcactaccctgactaagaacatcgccactctgggccctctgattctgcctctgtctgagaagttcctgttcttcgccaccttcgtggccaagaagctgctgaaggacaagatcaagcactactacgtgcccgacttcaaacttgccgtggaccacttttgcatccatgctggcggcagagctgttattgacgagctggagaagaaccttggcctgtctcccattgatgtggaggcctctcgatctacccttcaccgattcggcaacacctcttcttcttctatctggtacgagctggcctacatcgaagccaagggccgaatgaagaagggcaacaaggcctggcaaattgctctgggctctggcttcaagtgcaactctgccgtgtgggtggctctgagaaacgtgaaggcctctgccaattctccttggcagcactgcattgaccgataccccgtgaagatcgactctgacctgtctaagtctaagacccacgtgcagaacggccgatcttaa

SEQ ID NO: 95 - DNA, 1521 bp, artificial sequence
  gene BtFAE1
atgacctctgtgaacgtgaagctgatctaccactacgtgatcaccaacctgttcaacctgtgcttcttccccctgactgctatcgttgccggcaaagcttctcgactgaccattgacgacctgcaccacctgtactactcttacctgcagcacaacctgattaccatcgcccccctgtttgcctttaccgtgttcggctctgtgctgtacattgccacccgacctaagcctgtgtacctggtggagtactcttgttacctgccccccactcactgtcgatcttctatctctaaggtgatggacatcttctaccaggtgcgaaaggccgacccctctagaaatggcacctgcgacgactcttcttggctggacttcctgcgaaagatccaggagcgatctggcctgggagatgagactcatggccctgagggactgcttcacgtgcctcccagaaaaacctttgccgccgctagagaagaaaccgagaaggtgattatcggcgccctggagaacctgttcgagaacaccaaggtgaaccccaaggacatcggcatcctggtggtgaactcttctatgttcaaccccaccccctctctttctgccatggtggtgaacaccttcaagctgcgatctaacgtgcgatctttcaacctgggaggcatgggatgttctgctggcgtgatcgctattgacctggccaaagacctgctgcacgtgcacaagaacacctacgccctggtggtgtctaccgagaacatcacctacaacatctacgccggcgacaacaagtctatgatggtgtctaactgcctgttccgagtgggaggagccgctattctgctgtctaacaagccccgagaccgacgacgatctaagtacgagctggtgcacaccgtgcgaactcataccggagctgacgacaagtctttccgatgcgtgcaacagggcgatgacgagtctggaaagaccggcgtgtctctgtctaaggacatcaccgacgtggctggaagaaccgtgaagaagaacatctctaccctgggccctctgattctgcctctgtctgagaagctgctgttcttcgtgaccttcatgggcaagaagctgttcaaggacaagatcaagcactactacgtgcccgacttcaagcttgccatcgaccacttctgtatccacgctggcggacgagctgtgattgatgtgctggagaagaaccttggactggcccctattgatgtggaggcctctcgatctacccttcaccgattcggcaacacctcttcttcttctatctggtacgagctggcctacatcgaagctaagggccgaatgaagaagggcaacaaggtgtggcaaatcgctctgggctctggcttcaagtgcaactctgccgtttgggtggccctgagaaatgtgaaggcctctcgaaagtctccttgggagcactgcattgaccgataccccgtgaagatcgactacgactctgccaagtctgaggtgagagtgcagaacggccgatcttaa

SEQ ID NO: 96 - DNA, 1521 bp, artificial sequence
  gene CgKCS
atgacctctatcaacgtgaagctgctgtaccactacgtgctgaccaacttcttcaacctgtgcctgttccccctgactgcttttcctgccggcaaggcttctcaactgaccaccaacgacctgcaccacctgtactcttacctgcaccacaacctgatcaccgtgaccctgctgtttgccttcaccgtgttcggctctatcctgtacatcgtgaccagacccaagcctgtgtacctggtggactactcttgttacctgccccccagacatctgtcttgcggcatctctcgagtgatggagatcttctacgagatccgaaagtctgacccctctcgagaggtgcctttcgacgacccttcttctctggagttcctgcgaaagatccaggagcgatctggactgggagacgagacttatggaccccagggactggttcatgatatgcccctgcgaatgaattttgccgccgcccgagaagaaactgagcaggtgatcaacggagccctggagaagctgttcgagaacaccaaggtgaacccccgagagattggcatcctggtggtgaactcttctatgttcaaccccaccccctctctttctgccatggtggtgaacaccttcaagctgcgatctaacatcaagtctttctctctgggcggcatgggatgttctgccggcatcatcgctatcgacctggctaaggacctgctgcacgtgcacaagaacacctacgccctggtggtgtctaccgagaacatcacccactctacctacaccggcgacaaccgatctatgatggtgtctaactgcctgttcagaatgggcggagccgccattctgctgtctaacaaggctggcgaccgacgacgatctaagtacaagctggcccacactgtgagaactcacaccggcgctgacgatcagtctttccgatgcgtgcgacaggaggatgatgacagaggcaagatcggcgtgtgcctgtctaaagacatcaccgccgtggccggaaaaaccgtgaccaagaacatcgctaccctgggacctcttgtgctgcctctgtctgagaagttcctgtacgtggtgtctctgatggccaagaagctgttcaagaacaagatcaagcacacctacgtgcccgatttcaagctggccatcgaccacttctgcatccatgctggcggaagagctgtgattgacgtgctggagaagaacctggccctgtctcctgtggatgtggaggcttctcgatctaccctgcaccgattcggcaacacctcttcttcttctatctggtacgagctggcctacatcgaagccaagggccgaatgaagaagggcaacaaggtgtggcaaatcgccatcggctctggcttcaagtgcaactctgccgtttgggtggccctgtgtaatgtgaagccctctgtgaactctccttgggagcactgcattgacagataccccgtggagatcaactacggctcttctaagtctgagacccgagcccaaaacggccgatcttaa

SEQ ID NO: 97 - DNA, 804 bp, artificial sequence
  gene rELO2
atgaacatgtctgtgctgaccctgcaggagtacgagttcgagaagcagttcaacgagaacgaggccattcagtggatgcaggagaactggaagaagtccttcctgttctccgccctgtacgccgccttcattttcggcggccgacacctgatgaacaagcgagccaagttcgagctgcgaaagcccctggtcctgtggtctctgaccctggccgtcttctctatcttcggtgccctgcgaaccggtgcctacatgctgtacattctgatgaccaagggcctgaagcagtccgtctgtgaccagtccttctacaacggtcccgtctctaagttctgggcctacgccttcgtcctgtccaaggcccccgagctgggtgacaccattttcatcattctgcgaaagcagaagctgattttcctgcactggtaccaccacattaccgtcctgctgtactcctggtactcctacaaggacatggtcgccggcggtggctggttcatgaccatgaactacggcgtgcacgccgtcatgtactcctactacgccctgcgagccgccggcttccgagtctctcgaaagttcgccatgttcattaccctgtctcagattacccagatgctgatgggttgtgtcatcaactacctggtcttcaactggatgcagcacgacaacgaccagtgttactcccacttccagaacattttctggtcctccctgatgtacctgtcttacctgctgctgttctgccacttcttcttcgaggcctacattggtaaagtgaagaaggccaccaaggccgagtaa

SEQ ID NO: 98 - DNA, 972 bp, artificial sequence
  gene CpLCE
atgatcatcaagaacaacaacaacggctacttcattgacaacgtcaacaagatctgggagatccccatcaactctgagcacatggacatcctgaaggagatcccctggttcaagtacctgaccctgcccattgagcgaaactggaacggcatgaagctgttcctgtggaccaacgacaactactacctggcccacaccatctgcatcatctacgccttcttcatctacttcggtcccaagatcatggagaagcgaaagcccttcaagctggagaagcccctgaagtactggaacctgttcctggccctgttctctttcatcggcaccctgcgactgatgccctacgtgctgaccaacctgattaagtacggcttcgtctcttctatctgctccccccccattgcccccctgaccaagggccctgccggcctgtggctgtctctgttcatctattccaagtacattgagctgatcgacaccttcttcatcattgcccgaaagaagtctctgtccttcctgcactggttccaccacctgaccgtgctgctgtacacctgggacgcctacgtctgttgtcagaccattggtgtcttcttctgtgccattaactacttcgtgcactccatcatgtacttctactactacctgtcctcctgtggcaagcgacccaagtggggtatgatcattaccattctgcagatcgtccagatgattattggcaccattctgaccacctccggtatgtactactcttacaagcaccccttcgccaacgtgttccccgtcgagtacctgtcccagcccctgaaggtcggttgccacttcatccgaaccaacggtgtcttcgcctgcctgatgtacatctcttacttcgccctgttcttcgacttcttcatcaagcgatacatcaccaagggcacccccctggccgagtgggtcaccgctaacaagaagcccaccaagcgagactaa

SEQ ID NO: 99 - DNA, 795 bp, artificial sequence
  gene gELOVL6
atgtctgtgctgaccctgcaggagtacgagttcgagaagcagttcaacgagaacgaggccatccagtggatgcaggagaactggaagaagtctttcctgttctctgccctgtacgccgccttcgtcttcggcggccgacacctgatgaacaagcgagccaagttcgagctgcgaaagcccctggtgctgtggtctctgaccctggccgtgttctccattttcggcgccctgcgaaccggcgcctacatggtctacaccgtgatgaccaagggcctgaagcactccgtctgtgaccagggcttctacaacggccccgtctccaagttctgggcctacgccttcgtcctgtctaaggcccccgagctgggtgacaccatcttcattatcctgcgaaagcagaagctgattttcctgcactggtaccaccacattaccgtcctgctgtactcctggtactcctacaaggacatggtggccggcggtggttggttcatgaccatgaactactctgtgcactctgtgatgtactcctactacgccctgcgagccgccggcttccgagtctctcgaaagttcgccatgttcatcaccctgtcccagattctgcagatgctggtgggctgtgtcattaactacctggtgttccagtggatgcagcacgaccagtgccactcccacttccagaacatcttctggtcctctctgatgtacctgtcctacttcgtcctgttctgccacttcttcttcgaggcctacatcggctctaagatgcgaaaggccaccaaggccgactaa

SEQ ID NO: 100 - DNA, 1434 bp, artificial sequence
  gene D9DMB
atgtcctccgtggtcgagacctgtaagaccctgcccgtgcaggcctctcgactggtgcccaccgccgtcaaggaggaggtccccaccgaccacaacgtccccgacaactacgtgtcctggaccctgaagaaccagaagcccctgccccccatcgtgctggccaacctgctgcagaacatcgagtggctgaccttcatcattctgaccatcaccccctccatcgccatctacggtctgttcaccgtcaacatgcagtggaagaccttcgtgtggtctgtcatgtactacttcatcaccggcctgggcatcaccgccggctaccaccgactgtggtctcaccgatcctacaacgcctctaagcccctgcagtacttcctggccgtcgccggcaccggtgccgttgagggttccatcaagtggtggtgccgaaagcaccgagcccaccaccgatacaccgacaccgacctggacccctacaacgccaacaagggtttcttcttctcccacgtgggctggatgctggtcaagccccgagacaagcccggtgtggccgacatttctgacctgcgaaagtccgaggtcattcagtggcagcaccgatggtacgtgtggctgattgtgggtgccggtctgctgctgcccaccgtggtcgctggtctgggctggggagactgggccggtggtttcttctttgccggtgccgcccgactgaccttcgtgcaccactctaccttctgtgtcaactctctggcccactggctgggtgagacccccttcgacgacaagcactctccccgagaccacttcattaccgccctggtcaccgtgggcgagggctaccacaacttccaccaccagttccccatggactaccgaaacgccattcgatggtaccagtacgaccccaccaagtggttcatttggatgtgctccaagttcggcctggcctctcacctgaaggtcttccccgagaacgaggtgcgaaagggcgagctgaccatgcagctgaagaagctgcgagagacccaggacgtgctgacctgggcccccgacgtggagggactgcctgtgatttcttgggagtccttctctgagcagtccgtcacccgacccctgatcatcgtcgccggcttcatccacgacgtctctgacttcatcgacgagcaccccggtggccgacacctgattattaagtacattggtaaagacgccacccccgccttcttcggcggcgtttacgaccactccaacgccgcccacaacctgctgtccatgaagcgagtcggtgccctgcacggcggcatccagcacggactgcaggacatgtctattccccccgcccagcgactgcgaatcgcccgatacaacgagctggccggctctccctacaactcctctaccgccacctctgactctgagggtattctgggttaa

SEQ ID NO: 101 - DNA, 1020 bp, artificial sequence
  gene CeFAT6
atgaccgtcaagacccgatccaacattgccaagaagatcgagaaggacggtggccccgagacccagtacctggccgtggaccccaacgagatcattcagctgcaggaggagtctaagaagatcccctacaagatggagatcgtctggcgaaacgtggccctgttcgccgccctgcacttcgccgctgccatcggactgtaccagctgattttcgaggccaagtggcagaccgtgattttcaccttcctgctgtacgtcttcggtggtttcggcattaccgccggtgcccaccgactgtggtctcacaagtcctacaaggccaccacccccatgcgaattttcctgatgatcctgaacaacattgccctgcagaacgacgtcattgagtgggcccgagaccaccgatgtcaccacaagtggaccgacaccgacgccgacccccacaacaccacccgaggtttcttcttcgcccacatgggctggctgctggtgcgaaagcacccccaggtgaaggagcagggtgccaagctggacatgtccgacctgctgtctgaccccgtcctggtgttccagcgaaagcactacttccccctggtcatcctgtgttgtttcattctgcccaccattatccccgtctacttctggaaggagaccgccttcatcgccttctacaccgccggtaccttccgatactgcttcaccctgcacgccacctggtgtatcaactccgccgcccactacttcggttggaagccctacgactcctccattacccccgtggagaacgtgttcaccaccatcgccgccgtcggcgagggcggtcataacttccaccacaccttcccccaggactaccgaacctccgagtactctctgaagtacaactggacccgagtgctgatcgacaccgccgccgccctgggactggtgtacgaccgaaagaccgcctgtgacgagatcatcggccgacaggtgtctaaccacggctgtgacatccagcgaggtaaatctattatgtaa

SEQ ID NO: 102 - DNA, 1338 bp, artificial sequence
  gene MaOLE2
atggccacccccctgcctcctaccttcaccgtgcccgcctcctccaccgagacccgacgagaccccctgccccacgacgtgctgcctcctctgttcaacggtgagaaggtcaacatcctgaacatttggaagtacctggactggaagcacgtcatcggcctgctggtgacccccctggtcgccctttacggtatgtgtaccaccgagctgcacaccaagaccctggtctggtccatcgtgtactacttcgccaccggcctgggtatcaccgccggttaccaccgactgtgggcccaccgagcctacaacgccggtcccgctatgtccttcgccctggccctgttcggcgccggagctgttgagggctctatcaagtggtggtcccgaggccaccgagcccaccaccgatggaccgacaccgagaaggacccctactccgcccaccgaggtgtgttctactctcacctgggttggctgctgatcaagcgacccggttggaagattggtcacgccgacgtcgacgacctgaacaagaaccccctggtccagtggcagcacaagcactacctgatcctggtcattctgatgggtctggtgttccccaccgccgtcgccggtctgggatggggtgactggcgaggtggctacttctacgccgccattctgcgactgatcttcgtgcaccacgccaccttctgcgtgaactctctggcccactggctgggcgacggccctttcgacgaccgacacaccccccgagaccacttcatcaccgccttcctgaccctgggcgagggttaccacaacttccaccaccagttcccccaggactaccgatccgccatccgattctaccagtacgaccccaccaagtggctgattgccacctgcgccttcttcggtttcgcctctcacctgaagaccttccccgagaacgagattaagaagggcaagctgcagatgattgagaaggaggtgctggagaagaagaccaagctgcagtggggtacccccatcgccgacctgcccatcctgtccttcgaggacttccagcacgcctgcaagaacgaccgaaagcagtggatcctgctggagggcgtcgtctacgacgtcgccgacttcatgaccgagcaccccggtggcgagaagtacatcaagatgggcgtgggtaaagacatgacctccgccttcaacggcggtatgtacgaccactctaacgccgcccgaaacctgctgtctctgatgcgagtcgccgtcgtcgagttcggtggcgaggtcgaggcccagaagtcccgaccctctgtgaccgtgtacggcgaccactctaaggaggagtaa

SEQ ID NO: 103 - DNA, 918 bp, artificial sequence
  gene AtADS1
atgtctctgtctgcctctgagaaggaggagaacaacaagaagatggccgccgacaaggccgagatgggtcgaaagaagcgagccatgtgggagcgaaagtggaagcgactggacattgtgaaggccttcgcctccctgttcgtccacttcctgtgtctgctggcccccttcaacttcacctggcccgccctgcgagtggccctgattgtgtacaccgtgggtggcctgggcatcaccgtgtcttaccaccgaaacctggcccaccgatccttcaaggtccccaagtggctggagtacttcttcgcctactgcggcctgctggccattcagggcgaccccattgactgggtgtctacccaccgataccaccaccagttcaccgactccgaccgagacccccactcccccaacgagggtttctggttctctcacctgctgtggctgttcgacaccggctacctggtcgagaagtgcggccgacgaaccaacgtcgaggacctgaagcgacagtggtactacaagttcctgcagcgaaccgtcctgtaccacattctgaccttcggtttcctgctgtactacttcggtggtctgtctttcctgacctggggtatgggtattggtgtcgccatggagcaccacgtcacctgcctgattaactctctgtgtcacgtgtggggttctcgaacctggaagaccaacgacacctcccgaaacgtgtggtggctgtccgtgttctctttcggcgagtcctggcacaacaaccaccacgccttcgagtcctccgcccgacagggtctggagtggtggcagattgacatctcttggtacattgtccgattcctggagatcatcggcctggccaccgacgtgaagctgccctccgagtctcagcgacgacgaatggccatggtccgataa

SEQ ID NO: 104 - DNA, 924 bp, artificial sequence
  gene AtADS2
atgtctgtgacctctaccgtggaggagaaccaccagaagaacccctctacccctgctgctgtggaggaaaagaagaagcgacgatgggtgttctgggatcgacgatggcgacgactggactacgtgaagttctctgcctctttcaccgtgcactctctggctcttcttgcccccttctacttcacttggtctgccctgtgggtgaccttcctgttctacaccattggcggcctgggcattactgtgtcttaccaccgaaacctggcccaccgatctttcaaggtgcccaagtggctggaatacctgctggcttattgtgccctgctggccattcaaggtgaccctatcgactgggtgtctacccaccgataccaccaccagttcaccgactctgaacgagatccccactctcctaaagagggcttctggttctctcacctgctgtggatctacgactctgcctacctggtgtctaaatgcggccgacgagccaatgtggaggatctgaagcgacagtggttctaccgattcctgcagaagaccgtgctgttccacattcttggcctgggcttcttcctgttttacctgggcggcatgtcttttgtgacctggggaatgggagtgggagctgccctggaagttcatgtgacctgcctgatcaactctctgtgccacatctggggaacccgaacctggaaaaccaacgacacctctcgaaacgtgtggtggctgtctgtgttctctttcggcgagtcttggcacaacaaccaccacgccttcgagtcttctgctcgacagggactggaatggtggcagatcgacatctcttggtacatcgtgcgattcttcgagatcatcggcctggccaccgatgttaaagtgcccaccgaagcccaacgaagacgaatggccatcgtgagatga

SEQ ID NO: 105 - DNA, 1488 bp, artificial sequence
  gene EcAldH
atgaacttccaccacttggcttactggcaagacaaggctttgtctttggctatcgaaaacagattgttcatcaacggtgaatacactgctgctgctgaaaacgaaactttcgaaactgttgacccagttactcaagctccattggctaagatcgctagaggtaagtctgttgacatcgacagagctatgtctgctgctagaggtgttttcgaaagaggtgactggtctttgtcttctccagctaagagaaaggctgttttgaacaagttggctgacttgatggaagctcacgctgaagaattggctttgttggaaactttggacactggtaagccaatcagacactctttgagagacgacatcccaggtgctgctagagctatcagatggtacgctgaagctatcgacaaggtttacggtgaagttgctactacttcttctcacgaattggctatgatcgttagagaaccagttggtgttatcgctgctatcgttccatggaacttcccattgttgttgacttgttggaagttgggtccagctttggctgctggtaactctgttatcttgaagccatctgaaaagtctccattgtctgctatcagattggctggtttggctaaggaagctggtttgccagacggtgttttgaacgttgttactggtttcggtcacgaagctggtcaagctttgtctagacacaacgacatcgacgctatcgctttcactggttctactagaactggtaagcaattgttgaaggacgctggtgactctaacatgaagagagtttggttggaagctggtggtaagtctgctaacatcgttttcgctgactgtccagacttgcaacaagctgcttctgctactgctgctggtatcttctacaaccaaggtcaagtttgtatcgctggtactagattgttgttggaagaatctatcgctgacgaattcttggctttgttgaagcaacaagctcaaaactggcaaccaggtcacccattggacccagctactactatgggtactttgatcgactgtgctcacgctgactctgttcactctttcatcagagaaggtgaatctaagggtcaattgttgttggacggtagaaacgctggtttggctgctgctatcggtccaactatcttcgttgacgttgacccaaacgcttctttgtctagagaagaaatcttcggtccagttttggttgttactagattcacttctgaagaacaagctttgcaattggctaacgactctcaatacggtttgggtgctgctgtttggactagagacttgtctagagctcacagaatgtctagaagattgaaggctggttctgttttcgttaacaactacaacgacggtgacatgactgttccattcggtggttacaagcaatctggtaacggtagagacaagtctttgcacgctttggaaaagttcactgaattgaagactatctggatctctttggaagcttaa

SEQ ID NO: 106 - DNA, 1518 bp, artificial sequence
  gene ScZwf
atgagtgaaggccccgtcaaattcgaaaaaaataccgtcatatctgtctttggtgcgtcaggtgatctggcaaagaagaagacttttcccgccttatttgggcttttcagagaaggttaccttgatccatctaccaagatcttcggttatgcccggtccaaattgtccatggaggaggacctgaagtcccgtgtcctaccccacttgaaaaaacctcacggtgaagccgatgactctaaggtcgaacagttcttcaagatggtcagctacatttcgggaaattacgacacagatgaaggcttcgacgaattaagaacgcagatcgagaaattcgagaaaagtgccaacgtcgatgtcccacaccgtctcttctatctggccttgccgccaagcgtttttttgacggtggccaagcagatcaagagtcgtgtgtacgcagagaatggcatcacccgtgtaatcgtagagaaacctttcggccacgacctggcctctgccagggagctgcaaaaaaacctggggcccctctttaaagaagaagagttgtacagaattgaccattacttgggtaaagagttggtcaagaatcttttagtcttgaggttcggtaaccagtttttgaatgcctcgtggaatagagacaacattcaaagcgttcagatttcgtttaaagagaggttcggcaccgaaggccgtggcggctatttcgactctataggcataatcagagacgtgatgcagaaccatctgttacaaatcatgactctcttgactatggaaagaccggtgtcttttgacccggaatctattcgtgacgaaaaggttaaggttctaaaggccgtggcccccatcgacacggacgacgtcctcttgggccagtacggtaaatctgaggacgggtctaagcccgcctacgtggatgatgacactgtagacaaggactctaaatgtgtcacttttgcagcaatgactttcaacatcgaaaacgagcgttgggagggcgtccccatcatgatgcgtgccggtaaggctttgaatgagtccaaggtggagatcagactgcagtacaaagcggtcgcatcgggtgtcttcaaagacattccaaataacgaactggtcatcagagtgcagcccgatgccgctgtgtacctaaagtttaatgctaagacccctggtctgtcaaatgctacccaagtcacagatctgaatctaacttacgcaagcaggtaccaagacttttggattccagaggcttacgaggtgttgataagagacgccctactgggtgaccattccaactttgtcagagatgacgaattggatatcagttggggcatattcaccccattactgaagcacatagagcgtccggacggtccaacaccggaaatttacccctacggatcaagaggtccaaagggattgaaggaatatatgcaaaaacacaagtatgttatgcccgaaaagcacccttacgcttggcccgtgactaagccagaagatacgaaggataattag

SEQ ID NO: 107 - DNA, 1130 bp, Yarrowia lipolytica
  promoter gene GPAT
caacttttcttgtcgacctgagataccgaggttgcgcaggggatcaacttttgtgtctcagagggacccaagtgcgtacggagagtacagtacatactgtagctaacggtagcaggcgaactactggtacatacctcccccggaatatgtacaggcataatgcgtatctgtgggacatgtggtcgttgcgccattatgtaagcagcgtgtactcctctgactgtccatatggtttgctccatctcaccctcatcgttttcattgttcacaggcggccacaaaaaaactgtcttctctccttctctcttcgccttagtctactcggaccagttttagtttagcttggcgccactggataaatgagacctcaggccttgtgatgaggaggtcacttatgaagcatgttaggaggtgcttgtatggatagagaagcacccaaaataataagaataataataaaacagggggcgttgtcatttcatatcgtgttttcaccatcaatacacctccaaacaatgcccttcatgtggccagccccaatattgtcctgtagttcaactctatgcagctcgtatcttattgagcaagtaaaactctgtcagccgatattgcccgacccgcgacaagggtcaacaaggtggtgtaaggccttcgcagaagtcaaaactgtgccaaacaaacatctagagtctctttggtgtttctcgcatatatttaatcggctgtcttacgtatttggcctcggtaccggactaatttcggatcatccccaatacgctttttcttcgcagctgtcaacagtgtccatgatctatccacctaaatgggtcatatgaggcgtataatttcgtggtgctgataataattcccatatatttgacacaaaacttccccccctagacatacatctcacaatctcacttcttgtgcttctgtcacacatctcctccagctgacttcaactcacacctctgccccagttggtctacagcggtataaggtttctctgcatagaggtgcaccactcctcccgatacttgtttgtgtgacttgtgggtcacgacatatatatctacacacattgcgccaccctttggttcttccagcacaacaaaaacacgacacgctaa

SEQ ID NO: 108 - DNA, 522 bp, Yarrowia lipolytica
  promoter gene TEF1
agagaccgggttggcggcgcatttgtgtcccaaaaaacagccccaattgccccaattgaccccaaattgacccagtagcgggcccaaccccggcgagagcccccttctccccacatatcaaacctcccccggttcccacacttgccgttaagggcgtagggtactgcagtctggaatctacgcttgttcagactttgtactagtttctttgtctggccatccgggtaacccatgccggacgcaaaatagactactgaaaatttttttgctttgtggttgggactttagccaagggtataaaagaccaccgtccccgaattacctttcctcttcttttctctctctccttgtcaactcacacccgaaatcgttaagcatttccttctgagtataagaatcattcaaaatggtgagtttcagaggcagcagcaattgccacgggctttgagcacacggccgggtgtggtcccattcccatcgacacaagacgccacgtcatccgaccagcactttttgcagtac

SEQ ID NO: 109 - DNA, 1002 bp, Yarrowia lipolytica
  promoter gene EXP1
aaggagtttggcgcccgttttttcgagccccacacgtttcggtgagtatgagcggcggcagattcgagcgtttccggtttccgcggctggacgagagcccatgatgggggctcccaccaccagcaatcagggccctgattacacacccacctgtaatgtcatgctgttcatcgtggttaatgctgctgtgtgctgtgtgtgtgtgttgtttggcgctcattgttgcgttatgcagcgtacaccacaatattggaagcttattagcctttctattttttcgtttgcaaggcttaacaacattgctgtggagagggatggggatatggaggccgctggagggagtcggagaggcgttttggagcggcttggcctggcgcccagctcgcgaaacgcacctaggaccctttggcacgccgaaatgtgccacttttcagtctagtaacgccttacctacgtcattccatgcatgcatgtttgcgccttttttcccttgcccttgatcgccacacagtacagtgcactgtacagtggaggttttgggggggtcttagatgggagctaaaagcggcctagcggtacactagtgggattgtatggagtggcatggagcctaggtggagcctgacaggacgcacgaccggctagcccgtgacagacgatgggtggctcctgttgtccaccgcgtacaaatgtttgggccaaagtcttgtcagccttgcttgcgaacctaattcccaattttgtcacttcgcacccccattgatcgagccctaacccctgcccatcaggcaatccaattaagctcgcattgtctgccttgtttagtttggctcctgcccgtttcggcgtccacttgcacaaacacaaacaagcattatatataaggctcgtctctccctcccaaccacactcacttttttgcccgtcttcccttgctaacacaaaagtcaagaacacaaacaaccaccccaacccccttacacacaagacatatctacagca

SEQ ID NO: 110 - DNA, 438 bp, Yarrowia lipolytica
  promoter gene EYK1
tttgtgcaagtgtgtgtgtgtgtgtgtgtgtggtgtgtttgtgtgttagaacggatgttctggtgagtgtgagtgtgtagttgtgtgatgagaccttggtgccaccccaaggtatatatatataacacctccaggagctctaaaaaggcatctacttttctctatactgtacgtttcaatctggggaagcggaatcccaaaagggaaagccgccgcattaagctccacagccttgcataatccgatgacctgactagtgcggacaaagactattatttcgaggcaaggccaccacgtaccgcggtcccaaacttttgcaaagctgaaaacagcgtgggggtcaacgtggatcagaaagaggggcagatcagcttctataagaagctcctttccccacaattggcccacacgacacttctacacacttacacatctact

SEQ ID NO: 111 - DNA, 931 bp, Yarrowia lipolytica
  promoter gene GPD
cgcagtaggatgtcctgcacgggtctttttgtggggtgtggagaaaggggtgcttggagatggaagccggtagaaccgggctgcttggggggatttggggccgctgggctccaaagaggggtaggcatttcgttggggttacgtaattgcggcatttgggtcctgcgcgcatgtcccattggtcagaattagtccggataggagacttatcagccaatcacagcgccggatccacctgtaggttgggttgggtgggagcacccctccacagagtagagtcaaacagcagcagcaacatgatagttgggggtgtgcgtgttaaaggaaaaaaaaagaagcttgggttatattcccgctctatttagaggttgcgggatagacgccgacggagggcaatggcgccatggaaccttgcggatatcgatacgccgcggcggactgcgtccgaaccagctccagcagcgttttttccgggccattgagccgactgcgaccccgccaacgtgtcttggcccacgcactcatgtcatgttggtgttgggaggccactttttaagtagcacaaggcacctagctcgcagcaaggtgtccgaaccaaagaagcggctgcagtggtgcaaacggggcggaaacggcgggaaaaagccacgggggcacgaattgaggcacgccctcgaatttgagacgagtcacggccccattcgcccgcgcaatggctcgccaacgcccggtcttttgcaccacatcaggttaccccaagccaaacctttgtgttaaaaagcttaacatattataccgaacgtaggtttgggcgggcttgctccgtctgtccaaggcaacatttatataagggtctgcatcgccggctcaattgaatcttttttcttcttctcttctctatattcattcttgaattaaacacacatcaaca

SEQ ID NO: 112 - DNA, 407 bp, Yarrowia lipolytica
  terminator sequence XPR2
ccccacgttgccggtcttgcctcctactacctgtccatcaatgacgaggttctcacccctgcccaggtcgaggctcttattactgagtccaacaccggtgttcttcccaccaccaacctcaagggctctcccaacgctgttgcctacaacggtgttggcatttaggcaattaacagatagtttgccggtgataattctcttaacctcccacactcctttgacataacgatttatgtaacgaaactgaaatttgaccagatattgttgtaaatagaaaatctggcttgtaggtggcaaaatgcggcgtctttgttcatcaattccctctgtgactactcgtcatccctttatgttcgactgtcgtatttcttattttccatacatatgcaagtgagatgcccgtgtcc

SEQ ID NO: 113 - DNA, 500 bp, Yarrowia lipolytica
  terminator sequence LIP1t
ggttcatgagaagataaatatataaatacattgagatattaaatgcgctagattagagagcctcatactgctcggagagaagccaagacgagtactcaaaggggattacaccatccatatccacagacacaagctggggaaaggttctatatacactttccggaataccgtagtttccgatgttatcaatgggggcagccaggatttcaggcacttcggtgtctcggggtgaaatggcgttcttggcctccatcaagtcgtaccatgtcttcatttgcctgtcaaagtaaaacagaagcagatgaagaatgaacttgaagtgaaggacgtgactacaacagcctgcctggtcaaccacatcattcatgttgctgatgatcttctgaatcagctgaagagggtactctgtctcaatcagatcaccaaatttggggtgcagtagggcacatgatcgaagcatgagtgcagtagtagcacaataagtcattcgagcaaggtag

SEQ ID NO: 114 - DNA, 500 bp, Yarrowia lipolytica
  terminator sequence PQX3t
atggagcgtgtgttctgagtcgatgttttctatggagttgtgagtgttagtagacatgatgggtttatatatgatgaatgaatagatgtgattttgatttgcacgatggaattgagaactttgtaaacgtacatgggaatgtatgaatgtgggggttttgtgactggataactgacggtcagtggacgccgttgttcaaatatccaagagatgcgagaaactttgggtcaagtgaacatgtcctctctgttcaagtaaaccatcaactatgggtagtatatttagtaaggacaggagttgagagaggaaagttgccattctttggagtcccagaaacgtattttcgcgttccaagatcaaattagtagagtaatacgggcacgggaatccattcatagtctcaattttcccataggtgtgctacaaggtgttgagatgtggtacagtaccaccatgattcgagataaagagcccagaagtcattgatgaggtcaagaaat

SEQ ID NO: 115 - DNA, 1026 bp, artificial sequence
  Hygromycin (Hgr) resistance selection marker gene
atgaaaaagcctgaactcaccgccacgtctgtcgagaagtttctgatcgaaaagttcgacagcgtctccgacctgatgcagctctcggagggcgaagaatctcgtgctttcagcttcgatgtaggagggcgtggatatgtcctgcgggtaaatagctgcgccgatggtttctacaaagatcgttatgtttatcggcactttgcatcggccgcgctcccgattccggaagtgcttgacattggggaatttagcgagagcctgacctattgcatctcccgccgtgcacagggtgtcacgttgcaagacctgcctgaaaccgaactgcccgctgttctgcagccggtcgcggaggccatggatgcgatcgctgcggccgatcttagccagacgagcgggttcggcccattcggaccgcaaggaatcggtcaatacactacatggcgtgatttcatatgcgcgattgctgatccccatgtgtatcactggcaaactgtgatggacgacaccgtcagtgcgtccgtcgcgcaggctctcgatgagctgatgctttgggccgaggactgccccgaagtccggcacctcgtgcacgcggatttcggctccaacaatgtcctgacggacaatggccgcataacagcggtcattgactggagcgaggcgatgttcggggattcccaatacgaggtcgccaacatcttcttctggaggccgtggttggcttgtatggagcagcagacgcgctacttcgagcggaggcatccggagcttgcaggatcgccgcggctccgggcgtatatgctccgcattggtcttgaccaactctatcagagcttggttgacggcaatttcgatgatgcagcttgggcgcagggtcgatgcgacgcaatcgtccgatccggagccgggactgtcgggcgtacacaaatcgcccgcagaagcgcggccgtctggaccgatggctgtgtagaagtactcgccgatagtggaaaccgacgccccagcactcgtccgagggcaaaggaatag

SEQ ID NO: 116 - DNA, 1218 bp, Yarrowia lipolytica
  gene LEU
atggaacccgaaactaagaagaccaagactgactccaagaagattgttcttctcggcggcgacttctgtggccccgaggtgattgccgaggccgtcaaggtgctcaagtctgttgctgaggcctccggcaccgagtttgtgttcgaggaccgactcattggaggagctgccattgagaaggagggcgagcccatcaccgacgctactctcgacatctgccgaaaggctgactctattatgctcggtgctgtcggaggcgctgccaacaccgtatggaccactcccgacggacgaaccgacgtgcgacccgagcagggtctcctcaagctgcgaaaggacctgaacctgtacgccaacctgcgaccctgccagctgctgtcgcccaagctcgccgatctctcccccatccgaaacgttgagggcaccgacttcatcattgtccgagagctcgtcggaggtatctactttggagagcgaaaggaggatgacggatctggcgtcgcttccgacaccgagacctactccgttcctgaggttgagcgaattgcccgaatggccgccttcctggcccttcagcacaacccccctcttcccgtgtggtctcttgacaaggccaacgtgctggcctcctctcgactttggcgaaagactgtcactcgagtcctcaaggacgaattcccccagctcgagctcaaccaccagctgatcgactcggccgccatgatcctcatcaagcagccctccaagatgaatggtatcatcatcaccaccaacatgtttggcgatatcatctccgacgaggcctccgtcatccccggttctctgggtctgctgccctccgcctctctggcttctctgcccgacaccaacgaggcgttcggtctgtacgagccctgtcacggatctgcccccgatctcggcaagcagaaggtcaaccccattgccaccattctgtctgccgccatgatgctcaagttctctcttaacatgaagcccgccggtgacgctgttgaggctgccgtcaaggagtccgtcgaggctggtatcactaccgccgatatcggaggctcttcctccacctccgaggtcggagacttgttgccaacaaggtcaaggagctgctcaagaaggagtaagtcgtttctacgacgcattgatggaaggagcaaactgacgcgcctgcgggttggtctaccggcagggtccgctagtgtataa

SEQ ID NO: 117 - DNA, 855 bp, Yarrowia lipolytica
  gene URA3
atgccctcctacgaagctcgagctaacgtccacaagtccgcctttgccgctcgagtgctcaagctcgtggcagccaagaaaaccaacctgtgtgcttctctggatgttaccaccaccaaggagctcattgagcttgccgataaggtcggaccttatgtgtgcatgatcaaaacccatatcgacatcattgacgacttcacctacgccggcactgtgctccccctcaaggaacttgctcttaagcacggtttcttcctgttcgaggacagaaagttcgcagatattggcaacactgtcaagcaccagtaccggtgtcaccgaatcgccgagtggtccgatatcaccaacgcccacggtgtacccggaaccggaatcattgctggcctgcgagctggtgccgaggaaactgtctctgaacagaagaaggaggacgtctctgactacgagaactcccagtacaaggagttcctagtcccctctcccaacgagaagctggccagaggtctgctcatgctggccgagctgtcttgcaagggctctctggccactggcgagtactccaagcagaccattgagcttgcccgatccgaccccgagtttgtggttggcttcattgcccagaaccgacctaagggcgactctgaggactggcttattctgacccccggggtgggtcttgacgacaagggagacgctctcggacagcagtaccgaactgttgaggatgtcatgtctaccggaacggatatcataattgtcggccgaggtctgtacggccagaaccgagatcctattgaggaggccaagcgataccagaaggctggctgggaggcttaccagaagattaactgttag

SEQ ID NO: 118 - DNA, 619 bp, Yarrowia lipolytica
  homologous recombination fragment pex10-up
gtggtaatcgaccgactaaccatttttagctgacaaacacttgctaactcctataacgaatgaatgactaacttggcatattgttaccaagtattacttgggatatagttgagtgtaaccattgctaagaatccaaactggagcttctaaaggtctgggagtcgccgtatgtgttcatatcgaaatcaaagaaatcataatcgcaacagaattcaaaatcaagcagattaatatccattattgtactcggatcgtgacatatctgatatgatctcggatatgatctctgactgtttactgggagatttgttgaagatttgttgaggttatctgaaaagtagacaatagagacaaaatgacgatatcaagaactgaatcgggccgaaatactcggtatcattcccttcagcagtaactgtattgctctatcaatgcgacgagatacctccacaattaatactgtatacgctctaccactcatatctccaatgctaaaatatattcatgcccaggacctctgtgcactgctatgcagcacagtgttgtcgattgaattggtcgtgtctggtccctgatgctctgtgtctcgctgactagtccttccatccagacctcgtca

SEQ ID NO: 119 - DNA, 962 bp, Yarrowia lipolytica
  homologous recombination fragment pex10-dow
tttgagccgaggcagatttgggttgcttagtaagcagacgtggcgttgcaagtagatgtggcaaatggggacgaagattccgaggggatatcatagttccaaggggatgtcatcatttgccagctttcgccgccacttttgacgagtttttgtgggtcaaataagtttagttgaacttttcaaatttcagttggcattttgttaatagaaagggtgccggtgctggggggttcattcctcgggttgcagatatcctatctgtcttaggggtatctctttcaatcgacaagatgtagttgggtaacaattatttattaatattctctccatccagtacagtactaacatcttgacatctcagcacaagtgcatcttcccaagtgtttgttggagaggttgttgggtattacttaggaaacagaacacagtacgtggagatcttggatacatcgtacatggaggttatccataaaaaagaccctccaggactagttacaatgccgttagatgaggaaatccacaaccctgattcactatgaacatattatcttcccccaaacttgcgatatatggcccttgatgatagccttgattttacccttgatggtacctccacgaccaaccgatctgctgtttgaagagatattttcaaatttgaagtgctcagatctactaaacatgagtccagtaattctttccgtctttccgatttccgatattcccttttttagcccgacttttcactgctcccatgtcaaacgattaggacttgggagacaatcccactgtcaaaatcaccccgatattctctgtaaaacaagtacttcttccacgtgatcttcaaatacctcttccacgtgaccttcaaatacctcttcaagtacctcttccacgcgaccttcaaagtcccttcaaatacccttctcaattctccccttctcctccatagtccttctctctga

SEQ ID NO: 120 - DNA, 1134 bp, Yarrowia lipolytica
  pex10 gene
atgtggggaagttcacatgcattcgctggtgaatctgatctgacactacaactacacaccaggtccaacatgagcgacaatacgacaatcaaaaagccgatccgacccaaaccgatccggacggaacgcctgccttacgctggggccgcagaaatcatccgagccaaccagaaagaccactactttgagtccgtgcttgaacagcatctcgtcacgtttctgcagaaatggaagggagtacgatttatccaccagtacaaggaggagctggagacggcgtccaagtttgcatatctcggtttgtgtacgcttgtgggctccaagactctcggagaagagtacaccaatctcatgtacactatcagagaccgaacagctctaccgggggtggtgagacggtttggctacgtgctttccaacactctgtttccatacctgtttgtgcgctacatgggcaagttgcgcgccaaactgatgcgcgagtatccccatctggtggagtacgacgaagatgagcctgtgcccagcccggaaacatggaaggagcgggtcatcaagacgtttgtgaacaagtttgacaagttcacggcgctggaggggtttaccgcgatccacttggcgattttctacgtctacggctcgtactaccagctcagtaagcggatctggggcatgcgttatgtatttggacaccgactggacaagaatgagcctcgaatcggttacgagatgctcggtctgctgattttcgcccggtttgccacgtcatttgtgcagacgggaagagagtacctcggagcgctgctggaaaagagcgtggagaaagaggcaggggagaaggaagatgaaaaggaagcggttgtgccgaaaaagaagtcgtcaattccgttcattgaggatacagaaggggagacggaagacaagatcgatctggaggaccctcgacagctcaagttcattcctgaggcgtccagagcgtgcactctgtgtctgtcatacattagtgcgccggcatgtacgccatgtggacactttttctgttgggactgtatttccgaatgggtgagagagaagcccgagtgtcccttgtgtcggcagggtgtgagagagcagaacttgttgcctatcagataa

SEQ ID NO: 121 - DNA, 1533 bp, artificial sequence
  cardamine mustard CgKCSER gene
atgacctctatcaacgtgaagctgctgtaccactacgtgctgaccaacttcttcaacctgtgcctgttccccctgactgcttttcctgccggcaaggcttctcaactgaccaccaacgacctgcaccacctgtactcttacctgcaccacaacctgatcaccgtgaccctgctgtttgccttcaccgtgttcggctctatcctgtacatcgtgaccagacccaagcctgtgtacctggtggactactcttgttacctgccccccagacatctgtcttgcggcatctctcgagtgatggagatcttctacgagatccgaaagtctgacccctctcgagaggtgcctttcgacgacccttcttctctggagttcctgcgaaagatccaggagcgatctggactgggagacgagacttatggaccccagggactggttcatgatatgcccctgcgaatgaattttgccgccgcccgagaagaaactgagcaggtgatcaacggagccctggagaagctgttcgagaacaccaaggtgaacccccgagagattggcatcctggtggtgaactcttctatgttcaaccccaccccctctctttctgccatggtggtgaacaccttcaagctgcgatctaacatcaagtctttctctctgggcggcatgggatgttctgccggcatcatcgctatcgacctggctaaggacctgctgcacgtgcacaagaacacctacgccctggtggtgtctaccgagaacatcacccactctacctacaccggcgacaaccgatctatgatggtgtctaactgcctgttcagaatgggcggagccgccattctgctgtctaacaaggctggcgaccgacgacgatctaagtacaagctggcccacactgtgagaactcacaccggcgctgacgatcagtctttccgatgcgtgcgacaggaggatgatgacagaggcaagatcggcgtgtgcctgtctaaagacatcaccgccgtggccggaaaaaccgtgaccaagaacatcgctaccctgggacctcttgtgctgcctctgtctgagaagttcctgtacgtggtgtctctgatggccaagaagctgttcaagaacaagatcaagcacacctacgtgcccgatttcaagctggccatcgaccacttctgcatccatgctggcggaagagctgtgattgacgtgctggagaagaacctggccctgtctcctgtggatgtggaggcttctcgatctaccctgcaccgattcggcaacacctcttcttcttctatctggtacgagctggcctacatcgaagccaagggccgaatgaagaagggcaacaaggtgtggcaaatcgccatcggctctggcttcaagtgcaactctgccgtttgggtggccctgtgtaatgtgaagccctctgtgaactctccttgggagcactgcattgacagataccccgtggagatcaactacggctcttctaagtctgagacccgagcccaaaacggccgatctaaggacgagctgtaa

SEQ ID NO: 122 - DNA, 1557 bp, artificial sequence
  Yarrowia lipolytica DGAT1ER gene
atgactatcgactcacaatactacaagtcgcgagacaaaaacgacacggcacccaaaatcgcgggaatccgatatgccccgctatcgacaccattactcaaccgatgtgagaccttctctctggtctggcacattttcagcattcccactttcctcacaattttcatgctatgctgcgcaattccactgctctggccatttgtgattgcgtatgtagtgtacgctgttaaagacgactccccgtccaacggaggagtggtcaagcgatactcgcctatttcaagaaacttcttcatctggaagctctttggccgctacttccccataactctgcacaagacggtggatctggagcccacgcacacatactaccctctggacgtccaggagtatcacctgattgctgagagatactggccgcagaacaagtacctccgagcaatcatctccaccatcgagtactttctgcccgccttcatgaaacggtctctttctatcaacgagcaggagcagcctgccgagcgagatcctctcctgtctcccgtttctcccagctctccgggttctcaacctgacaagtggattaaccacgacagcagatatagccgtggagaatcatctggctccaacggccacgcctcgggctccgaacttaacggcaacggcaacaatggcaccactaaccgacgacctttgtcgtccgcctctgctggctccactgcatctgattccacgcttcttaacgggtccctcaactcctacgccaaccagatcattggcgaaaacgacccacagctgtcgcccacaaaactcaagcccactggcagaaaatacatcttcggctaccacccccacggcattatcggcatgggagcctttggtggaattgccaccgagggagctggatggtccaagctctttccgggcatccctgtttctcttatgactctcaccaacaacttccgagtgcctctctacagagagtacctcatgagtctgggagtcgcttctgtctccaagaagtcctgcaaggccctcctcaagcgaaaccagtctatctgcattgtcgttggtggagcacaggaaagtcttctggccagacccggtgtcatggacctggtgctactcaagcgaaagggttttgttcgacttggtatggaggtcggaaatgtcgcccttgttcccatcatggcctttggtgagaacgacctctatgaccaggttagcaacgacaagtcgtccaagctgtaccgattccagcagtttgtcaagaacttccttggattcacccttcctttgatgcatgcccgaggcgtcttcaactacgatgtcggtcttgtcccctacaggcgacccgtcaacattgtggttggttcccccattgacttgccttatctcccacaccccaccgacgaagaagtgtccgaataccacgaccgatacatcgccgagctgcagcgaatctacaacgagcacaaggatgaatatttcatcgattggaccgaggagggcaaaggagccccagagttccgaatgattgagaaggacgagctgtaa

SEQ ID NO: 123 - DNA, 1461 bp, artificial sequence
  Yarrowia lipolytica SCDER gene
atggtgaaaaacgtggaccaagtggatctctcgcaggtcgacaccattgcctccggccgagatgtcaactacaaggtcaagtacacctccggcgttaagatgagccagggcgcctacgacgacaagggccgccacatttccgagcagcccttcacctgggccaactggcaccagcacatcaactggctcaacttcattctggtgattgcgctgcctctgtcgtcctttgctgccgctcccttcgtctccttcaactggaagaccgccgcgtttgctgtcggctattacatgtgcaccggtctcggtatcaccgccggctaccaccgaatgtgggcccatcgagcctacaaggccgctctgcccgttcgaatcatccttgctctgtttggaggaggagctgtcgagggctccatccgatggtgggcctcgtctcaccgagtccaccaccgatggaccgactccaacaaggacccttacgacgcccgaaagggattctggttctcccactttggctggatgctgcttgtgcccaaccccaagaacaagggccgaactgacatttctgacctcaacaacgactgggttgtccgactccagcacaagtactacgtttacgttctcgtcttcatggccattgttctgcccaccctcgtctgtggctttggctggggcgactggaagggaggtcttgtctacgccggtatcatgcgatacacctttgtgcagcaggtgactttctgtgtcaactcccttgcccactggattggagagcagcccttcgacgaccgacgaactccccgagaccacgctcttaccgccctggtcacctttggagagggctaccacaacttccaccacgagttcccctcggactaccgaaacgccctcatctggtaccagtacgaccccaccaagtggctcatctggaccctcaagcaggttggtctcgcctgggacctccagaccttctcccagaacgccatcgagcagggtctcgtgcagcagcgacagaagaagctggacaagtggcgaaacaacctcaactggggtatccccattgagcagctgcctgtcattgagtttgaggagttccaagagcaggccaagacccgagatctggttctcatttctggcattgtccacgacgtgtctgcctttgtcgagcaccaccctggtggaaaggccctcattatgagcgccgtcggcaaggacggtaccgctgtcttcaacggaggtgtctaccgacactccaacgctggccacaacctgcttgccaccatgcgagtttcggtcattcgaggcggcatggaggttgaggtgtggaagactgcccagaacgaaaagaaggaccagaacattgtctccgatgagagtggaaaccgaatccaccgagctggtctccaggccacccgggtcgagaaccccggtatgtctggcatggctgctaaggacgagctgtag

SEQ ID NO: 124 - DNA, 1533 bp, artificial sequence
  Afican mustard BtFAE1ER gene
atgacctctgtgaacgtgaagctgatctaccactacgtgatcaccaacctgttcaacctgtgcttcttccccctgactgctatcgttgccggcaaagcttctcgactgaccattgacgacctgcaccacctgtactactcttacctgcagcacaacctgattaccatcgcccccctgtttgcctttaccgtgttcggctctgtgctgtacattgccacccgacctaagcctgtgtacctggtggagtactcttgttacctgccccccactcactgtcgatcttctatctctaaggtgatggacatcttctaccaggtgcgaaaggccgacccctctagaaatggcacctgcgacgactcttcttggctggacttcctgcgaaagatccaggagcgatctggcctgggagatgagactcatggccctgagggactgcttcacgtgcctcccagaaaaacctttgccgccgctagagaagaaaccgagaaggtgattatcggcgccctggagaacctgttcgagaacaccaaggtgaaccccaaggacatcggcatcctggtggtgaactcttctatgttcaaccccaccccctctctttctgccatggtggtgaacaccttcaagctgcgatctaacgtgcgatctttcaacctgggaggcatgggatgttctgctggcgtgatcgctattgacctggccaaagacctgctgcacgtgcacaagaacacctacgccctggtggtgtctaccgagaacatcacctacaacatctacgccggcgacaacaagtctatgatggtgtctaactgcctgttccgagtgggaggagccgctattctgctgtctaacaagccccgagaccgacgacgatctaagtacgagctggtgcacaccgtgcgaactcataccggagctgacgacaagtctttccgatgcgtgcaacagggcgatgacgagtctggaaagaccggcgtgtctctgtctaaggacatcaccgacgtggctggaagaaccgtgaagaagaacatctctaccctgggccctctgattctgcctctgtctgagaagctgctgttcttcgtgaccttcatgggcaagaagctgttcaaggacaagatcaagcactactacgtgcccgacttcaagcttgccatcgaccacttctgtatccacgctggcggacgagctgtgattgatgtgctggagaagaaccttggactggcccctattgatgtggaggcctctcgatctacccttcaccgattcggcaacacctcttcttcttctatctggtacgagctggcctacatcgaagctaagggccgaatgaagaagggcaacaaggtgtggcaaatcgctctgggctctggcttcaagtgcaactctgccgtttgggtggccctgagaaatgtgaaggcctctcgaaagtctccttgggagcactgcattgaccgataccccgtgaagatcgactacgactctgccaagtctgaggtgagagtgcagaacggccgatctaaggacgagctgtaa

SEQ ID NO: 125 - DNA, 1530 bp, artificial sequence
  cardamine mustard CgKCSPTS gene
atgacctctatcaacgtgaagctgctgtaccactacgtgctgaccaacttcttcaacctgtgcctgttccccctgactgcttttcctgccggcaaggcttctcaactgaccaccaacgacctgcaccacctgtactcttacctgcaccacaacctgatcaccgtgaccctgctgtttgccttcaccgtgttcggctctatcctgtacatcgtgaccagacccaagcctgtgtacctggtggactactcttgttacctgccccccagacatctgtcttgcggcatctctcgagtgatggagatcttctacgagatccgaaagtctgacccctctcgagaggtgcctttcgacgacccttcttctctggagttcctgcgaaagatccaggagcgatctggactgggagacgagacttatggaccccagggactggttcatgatatgcccctgcgaatgaattttgccgccgcccgagaagaaactgagcaggtgatcaacggagccctggagaagctgttcgagaacaccaaggtgaacccccgagagattggcatcctggtggtgaactcttctatgttcaaccccaccccctctctttctgccatggtggtgaacaccttcaagctgcgatctaacatcaagtctttctctctgggcggcatgggatgttctgccggcatcatcgctatcgacctggctaaggacctgctgcacgtgcacaagaacacctacgccctggtggtgtctaccgagaacatcacccactctacctacaccggcgacaaccgatctatgatggtgtctaactgcctgttcagaatgggcggagccgccattctgctgtctaacaaggctggcgaccgacgacgatctaagtacaagctggcccacactgtgagaactcacaccggcgctgacgatcagtctttccgatgcgtgcgacaggaggatgatgacagaggcaagatcggcgtgtgcctgtctaaagacatcaccgccgtggccggaaaaaccgtgaccaagaacatcgctaccctgggacctcttgtgctgcctctgtctgagaagttcctgtacgtggtgtctctgatggccaagaagctgttcaagaacaagatcaagcacacctacgtgcccgatttcaagctggccatcgaccacttctgcatccatgctggcggaagagctgtgattgacgtgctggagaagaacctggccctgtctcctgtggatgtggaggcttctcgatctaccctgcaccgattcggcaacacctcttcttcttctatctggtacgagctggcctacatcgaagccaagggccgaatgaagaagggcaacaaggtgtggcaaatcgccatcggctctggcttcaagtgcaactctgccgtttgggtggccctgtgtaatgtgaagccctctgtgaactctccttgggagcactgcattgacagataccccgtggagatcaactacggctcttctaagtctgagacccgagcccaaaacggccgatcttccaagctgtaa

SEQ ID NO: 126 - DNA, 1530 bp, artificial sequence
  African mustard BtFAE1PTS gene
atgacctctgtgaacgtgaagctgatctaccactacgtgatcaccaacctgttcaacctgtgcttcttccccctgactgctatcgttgccggcaaagcttctcgactgaccattgacgacctgcaccacctgtactactcttacctgcagcacaacctgattaccatcgcccccctgtttgcctttaccgtgttcggctctgtgctgtacattgccacccgacctaagcctgtgtacctggtggagtactcttgttacctgccccccactcactgtcgatcttctatctctaaggtgatggacatcttctaccaggtgcgaaaggccgacccctctagaaatggcacctgcgacgactcttcttggctggacttcctgcgaaagatccaggagcgatctggcctgggagatgagactcatggccctgagggactgcttcacgtgcctcccagaaaaacctttgccgccgctagagaagaaaccgagaaggtgattatcggcgccctggagaacctgttcgagaacaccaaggtgaaccccaaggacatcggcatcctggtggtgaactcttctatgttcaaccccaccccctctctttctgccatggtggtgaacaccttcaagctgcgatctaacgtgcgatctttcaacctgggaggcatgggatgttctgctggcgtgatcgctattgacctggccaaagacctgctgcacgtgcacaagaacacctacgccctggtggtgtctaccgagaacatcacctacaacatctacgccggcgacaacaagtctatgatggtgtctaactgcctgttccgagtgggaggagccgctattctgctgtctaacaagccccgagaccgacgacgatctaagtacgagctggtgcacaccgtgcgaactcataccggagctgacgacaagtctttccgatgcgtgcaacagggcgatgacgagtctggaaagaccggcgtgtctctgtctaaggacatcaccgacgtggctggaagaaccgtgaagaagaacatctctaccctgggccctctgattctgcctctgtctgagaagctgctgttcttcgtgaccttcatgggcaagaagctgttcaaggacaagatcaagcactactacgtgcccgacttcaagcttgccatcgaccacttctgtatccacgctggcggacgagctgtgattgatgtgctggagaagaaccttggactggcccctattgatgtggaggcctctcgatctacccttcaccgattcggcaacacctcttcttcttctatctggtacgagctggcctacatcgaagctaagggccgaatgaagaagggcaacaaggtgtggcaaatcgctctgggctctggcttcaagtgcaactctgccgtttgggtggccctgagaaatgtgaaggcctctcgaaagtctccttgggagcactgcattgaccgataccccgtgaagatcgactacgactctgccaagtctgaggtgagagtgcagaacggccgatcttccaagctgtaa

SEQ ID NO: 127 - DNA, 1596 bp, artificial sequence
  cardamine mustard CgKCSMTS
atgctttcactacgtcaatctataagatttttcaagccagccacaagaactttgtgtagctctagatatctgcttatgacctctatcaacgtgaagctgctgtaccactacgtgctgaccaacttcttcaacctgtgcctgttccccctgactgcttttcctgccggcaaggcttctcaactgaccaccaacgacctgcaccacctgtactcttacctgcaccacaacctgatcaccgtgaccctgctgtttgccttcaccgtgttcggctctatcctgtacatcgtgaccagacccaagcctgtgtacctggtggactactcttgttacctgccccccagacatctgtcttgcggcatctctcgagtgatggagatcttctacgagatccgaaagtctgacccctctcgagaggtgcctttcgacgacccttcttctctggagttcctgcgaaagatccaggagcgatctggactgggagacgagacttatggaccccagggactggttcatgatatgcccctgcgaatgaattttgccgccgcccgagaagaaactgagcaggtgatcaacggagccctggagaagctgttcgagaacaccaaggtgaacccccgagagattggcatcctggtggtgaactcttctatgttcaaccccaccccctctctttctgccatggtggtgaacaccttcaagctgcgatctaacatcaagtctttctctctgggcggcatgggatgttctgccggcatcatcgctatcgacctggctaaggacctgctgcacgtgcacaagaacacctacgccctggtggtgtctaccgagaacatcacccactctacctacaccggcgacaaccgatctatgatggtgtctaactgcctgttcagaatgggcggagccgccattctgctgtctaacaaggctggcgaccgacgacgatctaagtacaagctggcccacactgtgagaactcacaccggcgctgacgatcagtctttccgatgcgtgcgacaggaggatgatgacagaggcaagatcggcgtgtgcctgtctaaagacatcaccgccgtggccggaaaaaccgtgaccaagaacatcgctaccctgggacctcttgtgctgcctctgtctgagaagttcctgtacgtggtgtctctgatggccaagaagctgttcaagaacaagatcaagcacacctacgtgcccgatttcaagctggccatcgaccacttctgcatccatgctggcggaagagctgtgattgacgtgctggagaagaacctggccctgtctcctgtggatgtggaggcttctcgatctaccctgcaccgattcggcaacacctcttcttcttctatctggtacgagctggcctacatcgaagccaagggccgaatgaagaagggcaacaaggtgtggcaaatcgccatcggctctggcttcaagtgcaactctgccgtttgggtggccctgtgtaatgtgaagccctctgtgaactctccttgggagcactgcattgacagataccccgtggagatcaactacggctcttctaagtctgagacccgagcccaaaacggccgatcttaa